European Patent Application EP 4 357 457 A2, published April 24, 2024. Title: COMPOSITION FOR CLEAVING A TARGET DNA COMPRISING A GUIDE RNA SPECIFIC FOR THE TARGET DNA AND CAS PROTEIN-ENCODING NUCLEIC ACID OR CAS PROTEIN, AND USE THEREOF. Applicant: Toolgen Incorporated. Application EP. The sequence listing filed with the application follows.

SEQUENCE LISTING (296 sequences)

SEQ ID NO: 1 - DNA, 4107 bp, synthetic construct
  misc_feature 1..4107: note = Description of Artificial Sequence: Synthetic polynucleotide
  misc_feature 1..4107: note = Cas9-coding sequence
  source 1..4107: mol_type = other DNA
atggacaagaagtacagcatcggcctggacatcggtaccaacagcgtgggctgggccgtgatcaccgacgagtacaaggtgcccagcaagaagttcaaggtgctgggcaacaccgaccgccacagcatcaagaagaacctgatcggcgccctgctgttcgacagcggcgagaccgccgaggccacccgcctgaagcgcaccgcccgccgccgctacacccgccgcaagaaccgcatctgctacctgcaggagatcttcagcaacgagatggccaaggtggacgacagcttcttccaccgcctggaggagagcttcctggtggaggaggacaagaagcacgagcgccaccccatcttcggcaacatcgtggacgaggtggcctaccacgagaagtaccccaccatctaccacctgcgcaagaagctggtggacagcaccgacaaggccgacctgcgcctgatctacctggccctggcccacatgatcaagttccgcggccacttcctgatcgagggcgacctgaaccccgacaacagcgacgtggacaagctgttcatccagctggtgcagacctacaaccagctgttcgaggagaaccccatcaacgccagcggcgtggacgccaaggccatcctgagcgcccgcctgagcaagagccgccgcctggagaacctgatcgcccagctgcccggcgagaagaagaacggcctgttcggcaacctgatcgccctgagcctgggcctgacccccaacttcaagagcaacttcgacctggccgaggacgccaagctgcagctgagcaaggacacctacgacgacgacctggacaacctgctggcccagatcggcgaccagtacgccgacctgttcctggccgccaagaacctgagcgacgccatcctgctgagcgacatcctgcgcgtgaacaccgagatcaccaaggcccccctgagcgccagcatgatcaagcgctacgacgagcaccaccaggacctgaccctgctgaaggccctggtgcgccagcagctgcccgagaagtacaaggagatcttcttcgaccagagcaagaacggctacgccggctacatcgacggcggcgccagccaggaggagttctacaagttcatcaagcccatcctggagaagatggacggcaccgaggagctgctggtgaagctgaaccgcgaggacctgctgcgcaagcagcgcaccttcgacaacggcagcatcccccaccagatccacctgggcgagctgcacgccatcctgcgccgccaggaggacttctaccccttcctgaaggacaaccgcgagaagatcgagaagatcctgaccttccgcatcccctactacgtgggccccctggcccgcggcaacagccgcttcgcctggatgacccgcaagagcgaggagaccatcaccccctggaacttcgaggaggtggtggacaagggcgccagcgcccagagcttcatcgagcgcatgaccaacttcgacaagaacctgcccaacgagaaggtgctgcccaagcacagcctgctgtacgagtacttcaccgtgtacaacgagctgaccaaggtgaagtacgtgaccgagggcatgcgcaagcccgccttcctgagcggcgagcagaagaaggccatcgtggacctgctgttcaagaccaaccgcaaggtgaccgtgaagcagctgaaggaggactacttcaagaagatcgagtgcttcgacagcgtggagatcagcggcgtggaggaccgcttcaacgccagcctgggcacctaccacgacctgctgaagatcatcaaggacaaggacttcctggacaacgaggagaacgaggacatcctggaggacatcgtgctgaccctgaccctgttcgaggaccgcgagatgatcgaggagcgcctgaagacctacgcccacctgttcgacgacaaggtgatgaagcagctgaagcgccgccgctacaccggctggggccgcctgagccgcaagcttatcaacggcatccgcgacaagcagagcggcaagaccatcctggacttcctgaagagcgacggcttcgccaaccgcaacttcatgcagctgatccacgacgacagcctgaccttcaaggaggacatccagaaggcccaggtgagcggccagggcgacagcctgcacgagcacatcgccaacctggccggcagccccgccatcaagaagggcatcctgcagaccgtgaaggtggtggacgagctggtgaaggtgatgggccgccacaagcccgagaacatcgtgatcgagatggcccgcgagaaccagaccacccagaagggccagaagaacagccgcgagcgcatgaagcgcatcgaggagggcatcaaggagctgggcagccagatcctgaaggagcaccccgtggagaacacccagctgcagaacgagaagctgtacctgtactacctgcagaacggccgcgacatgtacgtggaccaggagctggacatcaaccgcctgagcgactacgacgtggaccacatcgtgccccagagcttcctgaaggacgacagcatcgacaacaaggtgctgacccgcagcgacaagaaccgcggcaagagcgacaacgtgcccagcgaggaggtggtgaagaagatgaagaactactggcgccagctgctgaacgccaagctgatcacccagcgcaagttcgacaacctgaccaaggccgagcgcggcggcctgagcgagctggacaaggccggcttcatcaagcgccagctggtggagacccgccagatcaccaagcacgtggcccagatcctggacagccgcatgaacaccaagtacgacgagaacgacaagctgatccgcgaggtgaaggtgatcaccctgaagagcaagctggtgagcgacttccgcaaggacttccagttctacaaggtgcgcgagatcaacaactaccaccacgcccacgacgcctacctgaacgccgtggtgggcaccgccctgatcaagaagtaccccaagctggagagcgagttcgtgtacggcgactacaaggtgtacgacgtgcgcaagatgatcgccaagagcgagcaggagatcggcaaggccaccgccaagtacttcttctacagcaacatcatgaacttcttcaagaccgagatcaccctggccaacggcgagatccgcaagcgccccctgatcgagaccaacggcgagaccggcgagatcgtgtgggacaagggccgcgacttcgccaccgtgcgcaaggtgctgagcatgccccaggtgaacatcgtgaagaagaccgaggtgcagaccggcggcttcagcaaggagagcatcctgcccaagcgcaacagcgacaagctgatcgcccgcaagaaggactgggaccccaagaagtacggcggcttcgacagccccaccgtggcctacagcgtgctggtggtggccaaggtggagaagggcaagagcaagaagctgaagagcgtgaaggagctgctgggcatcaccatcatggagcgcagcagcttcgagaagaaccccatcgacttcctggaggccaagggctacaaggaggtgaagaaggacctgatcatcaagctgcccaagtacagcctgttcgagctggagaacggccgcaagcgcatgctggccagcgccggcgagctgcagaagggcaacgagctggccctgcccagcaagtacgtgaacttcctgtacctggccagccactacgagaagctgaagggcagccccgaggacaacgagcagaagcagctgttcgtggagcagcacaagcactacctggacgagatcatcgagcagatcagcgagttcagcaagcgcgtgatcctggccgacgccaacctggacaaggtgctgagcgcctacaacaagcaccgcgacaagcccatccgcgagcaggccgagaacatcatccacctgttcaccctgaccaacctgggcgcccccgccgccttcaagtacttcgacaccaccatcgaccgcaagcgctacaccagcaccaaggaggtgctggacgccaccctgatccaccagagcatcaccggtctgtacgagacccgcatcgacctgagccagctgggcggcgactaa

SEQ ID NO: 2 - protein, 21 aa, synthetic construct
  REGION 1..21: note = Description of Artificial Sequence: Synthetic peptide
  REGION 1..21: note = Peptide tag
GGSGPPKKKRKVYPYDVPDYA

SEQ ID NO: 3 - DNA, 34 bp, synthetic construct
  misc_feature 1..34: note = Description of Artificial Sequence: Synthetic oligonucleotide
  misc_feature 1..34: note = F primer for CCR5
  source 1..34: mol_type = other DNA
aattcatgacatcaattattatacatcggaggag

SEQ ID NO: 4 - DNA, 34 bp, synthetic construct
  misc_feature 1..34: note = Description of Artificial Sequence: Synthetic oligonucleotide
  misc_feature 1..34: note = R primer for CCR5
  source 1..34: mol_type = other DNA
gatcctcctccgatgtataataattgatgtcatg

SEQ ID NO: 5 - DNA, 20 bp, synthetic construct
  misc_feature 1..20: note = Description of Artificial Sequence: Synthetic oligonucleotide
  misc_feature 1..20: note = F1 primer for CCR5
  source 1..20: mol_type = other DNA
ctccatggtgctatagagca

SEQ ID NO: 6 - DNA, 21 bp, synthetic construct
  misc_feature 1..21: note = Description of Artificial Sequence: Synthetic oligonucleotide
  misc_feature 1..21: note = F2 primer for CCR5
  source 1..21: mol_type = other DNA
gagccaagctctccatctagt

SEQ ID NO: 7 - DNA, 20 bp, synthetic construct
  misc_feature 1..20: note = Description of Artificial Sequence: Synthetic oligonucleotide
  misc_feature 1..20: note = R primer for CCR5
  source 1..20: mol_type = other DNA
gccctgtcaagagttgacac

SEQ ID NO: 8 - DNA, 20 bp, synthetic construct
  misc_feature 1..20: note = Description of Artificial Sequence: Synthetic oligonucleotide
  misc_feature 1..20: note = F1 primer for C4BPB
  source 1..20: mol_type = other DNA
tatttggctggttgaaaggg

SEQ ID NO: 9 - DNA, 24 bp, synthetic construct
  misc_feature 1..24: note = Description of Artificial Sequence: Synthetic oligonucleotide
  misc_feature 1..24: note = R1 primer for C4BPB
  source 1..24: mol_type = other DNA
aaagtcatgaaataaacacaccca

SEQ ID NO: 10 - DNA, 24 bp, synthetic construct
  misc_feature 1..24: note = Description of Artificial Sequence: Synthetic oligonucleotide
  misc_feature 1..24: note = F2 primer for C4BPB
  source 1..24: mol_type = other DNA
ctgcattgatatggtagtaccatg

SEQ ID NO: 11 - DNA, 21 bp, synthetic construct
  misc_feature 1..21: note = Description of Artificial Sequence: Synthetic oligonucleotide
  misc_feature 1..21: note = R2 primer for C4BPB
  source 1..21: mol_type = other DNA
gctgttcattgcaatggaatg

SEQ ID NO: 12 - DNA, 20 bp, synthetic construct
  misc_feature 1..20: note = Description of Artificial Sequence: Synthetic oligonucleotide
  misc_feature 1..20: note = F1 primer for ADCY5
  source 1..20: mol_type = other DNA
gctcccaccttagtgctctg

SEQ ID NO: 13 - DNA, 20 bp, synthetic construct
  misc_feature 1..20: note = Description of Artificial Sequence: Synthetic oligonucleotide
  misc_feature 1..20: note = R1 primer for ADCY5
  source 1..20: mol_type = other DNA
ggtggcaggaacctgtatgt

SEQ ID NO: 14 - DNA, 21 bp, synthetic construct
  misc_feature 1..21: note = Description of Artificial Sequence: Synthetic oligonucleotide
  misc_feature 1..21: note = F2 primer for ADCY5
  source 1..21: mol_type = other DNA
gtcattggccagagatgtgga

SEQ ID NO: 15 - DNA, 20 bp, synthetic construct
  misc_feature 1..20: note = Description of Artificial Sequence: Synthetic oligonucleotide
  misc_feature 1..20: note = R2 primer for ADCY5
  source 1..20: mol_type = other DNA
gtcccatgacaggcgtgtat

SEQ ID NO: 16 - DNA, 20 bp, synthetic construct
  misc_feature 1..20: note = Description of Artificial Sequence: Synthetic oligonucleotide
  misc_feature 1..20: note = F primer for KCNJ6
  source 1..20: mol_type = other DNA
gcctggccaagtttcagtta

SEQ ID NO: 17 - DNA, 20 bp, synthetic construct
  misc_feature 1..20: note = Description of Artificial Sequence: Synthetic oligonucleotide
  misc_feature 1..20: note = R1 primer for KCNJ6
  source 1..20: mol_type = other DNA
tggagccattggtttgcatc

SEQ ID NO: 18 - DNA, 22 bp, synthetic construct
  misc_feature 1..22: note = Description of Artificial Sequence: Synthetic oligonucleotide
  misc_feature 1..22: note = R2 primer for KCNJ6
  source 1..22: mol_type = other DNA
ccagaactaagccgtttctgac

SEQ ID NO: 19 - DNA, 20 bp, synthetic construct
  misc_feature 1..20: note = Description of Artificial Sequence: Synthetic oligonucleotide
  misc_feature 1..20: note = F1 primer for CNTNAP2
  source 1..20: mol_type = other DNA
atcaccgacaaccagtttcc

SEQ ID NO: 20 - DNA, 20 bp, synthetic construct
  misc_feature 1..20: note = Description of Artificial Sequence: Synthetic oligonucleotide
  misc_feature 1..20: note = F2 primer for CNTNAP2
  source 1..20: mol_type = other DNA
tgcagtgcagactctttcca

SEQ ID NO: 21 - DNA, 20 bp, synthetic construct
  misc_feature 1..20: note = Description of Artificial Sequence: Synthetic oligonucleotide
  misc_feature 1..20: note = R primer for CNTNAP2
  source 1..20: mol_type = other DNA
aaggacacagggcaactgaa

SEQ ID NO: 22 - DNA, 20 bp, synthetic construct
  misc_feature 1..20: note = Description of Artificial Sequence: Synthetic oligonucleotide
  misc_feature 1..20: note = F1 primer for N/A Chr. 5
  source 1..20: mol_type = other DNA
tgtggaacgagtggtgacag

SEQ ID NO: 23 - DNA, 22 bp, synthetic construct
  misc_feature 1..22: note = Description of Artificial Sequence: Synthetic oligonucleotide
  misc_feature 1..22: note = R1 primer for N/A Chr. 5
  source 1..22: mol_type = other DNA
gctggattaggaggcaggattc

SEQ ID NO: 24 - DNA, 22 bp, synthetic construct
  misc_feature 1..22: note = Description of Artificial Sequence: Synthetic oligonucleotide
  misc_feature 1..22: note = F2 primer for N/A Chr. 5
  source 1..22: mol_type = other DNA
gtgctgagaacgcttcatagag

SEQ ID NO: 25 - DNA, 23 bp, synthetic construct
  misc_feature 1..23: note = Description of Artificial Sequence: Synthetic oligonucleotide
  misc_feature 1..23: note = R2 primer for N/A Chr. 5
  source 1..23: mol_type = other DNA
ggaccaaaccacattcttctcac

SEQ ID NO: 26 - DNA, 20 bp, synthetic construct
  misc_feature 1..20: note = Description of Artificial Sequence: Synthetic oligonucleotide
  misc_feature 1..20: note = F primer for deletion
  source 1..20: mol_type = other DNA
ccacatctcgttctcggttt

SEQ ID NO: 27 - DNA, 20 bp, synthetic construct
  misc_feature 1..20: note = Description of Artificial Sequence: Synthetic oligonucleotide
  misc_feature 1..20: note = R primer for deletion
  source 1..20: mol_type = other DNA
tcacaagcccacagatattt

SEQ ID NO: 28 - RNA, 105 nt, synthetic construct
  misc_feature 1..105: note = Description of Artificial Sequence: Synthetic polynucleotide
  misc_feature 1..105: note = sgRNA for CCR5
  source 1..105: mol_type = other RNA
ggtgacatcaattattatacatgttttagagctagaaatagcaagttaaaataaggctagtccgttatcaacttgaaaaagtggcaccgagtcggtgcttttttt

SEQ ID NO: 29 - RNA, 44 nt, synthetic construct
  misc_feature 1..44: note = Description of Artificial Sequence: Synthetic oligonucleotide
  misc_feature 1..44: note = crRNA for CCR5
  source 1..44: mol_type = other RNA
ggtgacatcaattattatacatgttttagagctatgctgttttg

SEQ ID NO: 30 - RNA, 86 nt, synthetic construct
  misc_feature 1..86: note = Description of Artificial Sequence: Synthetic oligonucleotide
  misc_feature 1..86: note = tracrRNA for CCR5
  source 1..86: mol_type = other RNA
ggaaccattcaaaacagcatagcaagttaaaataaggctagtccgttatcaacttgaaaaagtggcaccgagtcggtgcttttttt

SEQ ID NO: 31 - DNA, 86 bp, synthetic construct
  misc_feature 1..86: note = Description of Artificial Sequence: Synthetic oligonucleotide
  misc_feature 1..86: note = Foxn1 #1 sgRNA
  source 1..86: mol_type = other DNA
gaaattaatacgactcactataggcagtctgacgtcacacttccgttttagagctagaaatagcaagttaaaataaggctagtccg

SEQ ID NO: 32 - DNA, 86 bp, synthetic construct
  misc_feature 1..86: note = Description of Artificial Sequence: Synthetic oligonucleotide
  misc_feature 1..86: note = Foxn1 #2 sgRNA
  source 1..86: mol_type = other DNA
gaaattaatacgactcactataggacttccaggctccacccgacgttttagagctagaaatagcaagttaaaataaggctagtccg

SEQ ID NO: 33 - DNA, 86 bp, synthetic construct
  misc_feature 1..86: note = Description of Artificial Sequence: Synthetic oligonucleotide
  misc_feature 1..86: note = Foxn1 #3 sgRNA
  source 1..86: mol_type = other DNA
gaaattaatacgactcactataggccaggctccacccgactggagttttagagctagaaatagcaagttaaaataaggctagtccg

SEQ ID NO: 34 - DNA, 86 bp, synthetic construct
  misc_feature 1..86: note = Description of Artificial Sequence: Synthetic oligonucleotide
  misc_feature 1..86: note = Foxn1 #4 sgRNA
  source 1..86: mol_type = other DNA
gaaattaatacgactcactataggactggagggcgaaccccaaggttttagagctagaaatagcaagttaaaataaggctagtccg

SEQ ID NO: 35 - DNA, 86 bp, synthetic construct
  misc_feature 1..86: note = Description of Artificial Sequence: Synthetic oligonucleotide
  misc_feature 1..86: note = Foxn1 #5 sgRNA
  source 1..86: mol_type = other DNA
gaaattaatacgactcactataggaccccaaggggacctcatgcgttttagagctagaaatagcaagttaaaataaggctagtccg

SEQ ID NO: 36 - DNA, 86 bp, synthetic construct
  misc_feature 1..86: note = Description of Artificial Sequence: Synthetic oligonucleotide
  misc_feature 1..86: note = Prkdc #1 sgRNA
  source 1..86: mol_type = other DNA
gaaattaatacgactcactataggttagttttttccagagacttgttttagagctagaaatagcaagttaaaataaggctagtccg

SEQ ID NO: 37 - DNA, 86 bp, synthetic construct
  misc_feature 1..86: note = Description of Artificial Sequence: Synthetic oligonucleotide
  misc_feature 1..86: note = Prkdc #2 sgRNA
  source 1..86: mol_type = other DNA
gaaattaatacgactcactataggttggtttgcttgtgtttatcgttttagagctagaaatagcaagttaaaataaggctagtccg

SEQ ID NO: 38 - DNA, 86 bp, synthetic construct
  misc_feature 1..86: note = Description of Artificial Sequence: Synthetic oligonucleotide
  misc_feature 1..86: note = Prkdc #3 sgRNA
  source 1..86: mol_type = other DNA
gaaattaatacgactcactataggcacaagcaaaccaaagtctcgttttagagctagaaatagcaagttaaaataaggctagtccg

SEQ ID NO: 39 - DNA, 86 bp, synthetic construct
  misc_feature 1..86: note = Description of Artificial Sequence: Synthetic oligonucleotide
  misc_feature 1..86: note = Prkdc #4 sgRNA
  source 1..86: mol_type = other DNA
gaaattaatacgactcactataggcctcaatgctaagcgacttcgttttagagctagaaatagcaagttaaaataaggctagtccg

SEQ ID NO: 40 - DNA, 29 bp, synthetic construct
  misc_feature 1..29: note = Description of Artificial Sequence: Synthetic oligonucleotide
  misc_feature 1..29: note = F1 primer for Foxn1
  source 1..29: mol_type = other DNA
gtctgtctatcatctcttcccttctctcc

SEQ ID NO: 41 - DNA, 25 bp, synthetic construct
  misc_feature 1..25: note = Description of Artificial Sequence: Synthetic oligonucleotide
  misc_feature 1..25: note = F2 primer for Foxn1
  source 1..25: mol_type = other DNA
tccctaatccgatggctagctccag

SEQ ID NO: 42 - DNA, 23 bp, synthetic construct
  misc_feature 1..23: note = Description of Artificial Sequence: Synthetic oligonucleotide
  misc_feature 1..23: note = R1 primer for Foxn1
  source 1..23: mol_type = other DNA
acgagcagctgaagttagcatgc

SEQ ID NO: 43 - DNA, 32 bp, synthetic construct
  misc_feature 1..32: note = Description of Artificial Sequence: Synthetic oligonucleotide
  misc_feature 1..32: note = R2 primer for Foxn1
  source 1..32: mol_type = other DNA
ctactcaatgctcttagagctaccaggcttgc

SEQ ID NO: 44 - DNA, 20 bp, synthetic construct
  misc_feature 1..20: note = Description of Artificial Sequence: Synthetic oligonucleotide
  misc_feature 1..20: note = F primer for Prkdc
  source 1..20: mol_type = other DNA
gactgttgtggggagggccg

SEQ ID NO: 45 - DNA, 24 bp, synthetic construct
  misc_feature 1..24: note = Description of Artificial Sequence: Synthetic oligonucleotide
  misc_feature 1..24: note = F2 primer for Prkdc
  source 1..24: mol_type = other DNA
gggagggccgaaagtcttattttg

SEQ ID NO: 46 - DNA, 28 bp, synthetic construct
  misc_feature 1..28: note = Description of Artificial Sequence: Synthetic oligonucleotide
  misc_feature 1..28: note = R1 primer for Prkdc
  source 1..28: mol_type = other DNA
cctgaagactgaagttggcagaagtgag

SEQ ID NO: 47 - DNA, 27 bp, synthetic construct
  misc_feature 1..27: note = Description of Artificial Sequence: Synthetic oligonucleotide
  misc_feature 1..27: note = R2 primer for Prkdc
  source 1..27: mol_type = other DNA
ctttagggcttcttctctacaatcacg

SEQ ID NO: 48 - DNA, 38 bp, synthetic construct
  misc_feature 1..38: note = Description of Artificial Sequence: Synthetic oligonucleotide
  misc_feature 1..38: note = F primer for Foxn1
  source 1..38: mol_type = other DNA
ctcggtgtgtagccctgacctcggtgtgtagccctgac

SEQ ID NO: 49 - DNA, 21 bp, synthetic construct
  misc_feature 1..21: note = Description of Artificial Sequence: Synthetic oligonucleotide
  misc_feature 1..21: note = R primer for Foxn1
  source 1..21: mol_type = other DNA
agactggcctggaactcacag

SEQ ID NO: 50 - DNA, 23 bp, synthetic construct
  misc_feature 1..23: note = Description of Artificial Sequence: Synthetic oligonucleotide
  misc_feature 1..23: note = F primer for Foxn1
  source 1..23: mol_type = other DNA
cactaaagcctgtcaggaagccg

SEQ ID NO: 51 - DNA, 21 bp, synthetic construct
  misc_feature 1..21: note = Description of Artificial Sequence: Synthetic oligonucleotide
  misc_feature 1..21: note = R primer for Foxn1
  source 1..21: mol_type = other DNA
ctgtggagagcacacagcagc

SEQ ID NO: 52 - DNA, 19 bp, synthetic construct
  misc_feature 1..19: note = Description of Artificial Sequence: Synthetic oligonucleotide
  misc_feature 1..19: note = F primer for Foxn1
  source 1..19: mol_type = other DNA
gctgcgacctgagaccatg

SEQ ID NO: 53 - DNA, 26 bp, synthetic construct
  misc_feature 1..26: note = Description of Artificial Sequence: Synthetic oligonucleotide
  misc_feature 1..26: note = R primer for Foxn1
  source 1..26: mol_type = other DNA
cttcaatggcttcctgcttaggctac

SEQ ID NO: 54 - DNA, 23 bp, synthetic construct
  misc_feature 1..23: note = Description of Artificial Sequence: Synthetic oligonucleotide
  misc_feature 1..23: note = F primer for Foxn1
  source 1..23: mol_type = other DNA
ggttcagatgaggccatcctttc

SEQ ID NO: 55 - DNA, 24 bp, synthetic construct
  misc_feature 1..24: note = Description of Artificial Sequence: Synthetic oligonucleotide
  misc_feature 1..24: note = R primer for Foxn1
  source 1..24: mol_type = other DNA
cctgatctgcaggcttaacccttg

SEQ ID NO: 56 - DNA, 22 bp, synthetic construct
  misc_feature 1..22: note = Description of Artificial Sequence: Synthetic oligonucleotide
  misc_feature 1..22: note = F primer for Prkdc
  source 1..22: mol_type = other DNA
ctcacctgcacatcacatgtgg

SEQ ID NO: 57 - DNA, 20 bp, synthetic construct
  misc_feature 1..20: note = Description of Artificial Sequence: Synthetic oligonucleotide
  misc_feature 1..20: note = R primer for Prkdc
  source 1..20: mol_type = other DNA
ggcatccaccctatggggtc

SEQ ID NO: 58 - DNA, 25 bp, synthetic construct
  misc_feature 1..25: note = Description of Artificial Sequence: Synthetic oligonucleotide
  misc_feature 1..25: note = F primer for Prkdc
  source 1..25: mol_type = other DNA
gccttgacctagagcttaaagagcc

SEQ ID NO: 59 - DNA, 25 bp, synthetic construct
  misc_feature 1..25: note = Description of Artificial Sequence: Synthetic oligonucleotide
  misc_feature 1..25: note = R primer for Prkdc
  source 1..25: mol_type = other DNA
ggtcttgttagcaggaaggacactg

SEQ ID NO: 60 - DNA, 27 bp, synthetic construct
  misc_feature 1..27: note = Description of Artificial Sequence: Synthetic oligonucleotide
  misc_feature 1..27: note = F primer for Prkdc
  source 1..27: mol_type = other DNA
aaaactctgcttgatgggatatgtggg

SEQ ID NO: 61 - DNA, 26 bp, synthetic construct
  misc_feature 1..26: note = Description of Artificial Sequence: Synthetic oligonucleotide
  misc_feature 1..26: note = R primer for Prkdc
  source 1..26: mol_type = other DNA
ctctcactggttatctgtgctccttc

SEQ ID NO: 62 - DNA, 23 bp, synthetic construct
  misc_feature 1..23: note = Description of Artificial Sequence: Synthetic oligonucleotide
  misc_feature 1..23: note = F primer for Prkdc
  source 1..23: mol_type = other DNA
ggatcaataggtggtgggggatg

SEQ ID NO: 63 - DNA, 27 bp, synthetic construct
  misc_feature 1..27: note = Description of Artificial Sequence: Synthetic oligonucleotide
  misc_feature 1..27: note = R primer for Prkdc
  source 1..27: mol_type = other DNA
gtgaatgacacaatgtgacagcttcag

SEQ ID NO: 64 - DNA, 28 bp, synthetic construct
  misc_feature 1..28: note = Description of Artificial Sequence: Synthetic oligonucleotide
  misc_feature 1..28: note = F primer for Prkdc
  source 1..28: mol_type = other DNA
cacaagacagacctctcaacattcagtc

SEQ ID NO: 65 - DNA, 32 bp, synthetic construct
  misc_feature 1..32: note = Description of Artificial Sequence: Synthetic oligonucleotide
  misc_feature 1..32: note = R primer for Prkdc
  source 1..32: mol_type = other DNA
gtgcatgcatataatccattctgattgctctc

SEQ ID NO: 66 - DNA, 17 bp, synthetic construct
  misc_feature 1..17: note = Description of Artificial Sequence: Synthetic oligonucleotide
  misc_feature 1..17: note = F1 primer for Prkdc
  source 1..17: mol_type = other DNA
gggaggcagaggcaggt

SEQ ID NO: 67 - DNA, 23 bp, synthetic construct
  misc_feature 1..23: note = Description of Artificial Sequence: Synthetic oligonucleotide
  misc_feature 1..23: note = F2 primer for Prkdc
  source 1..23: mol_type = other DNA
ggatctctgtgagtttgaggcca

SEQ ID NO: 68 - DNA, 24 bp, synthetic construct
  misc_feature 1..24: note = Description of Artificial Sequence: Synthetic oligonucleotide
  misc_feature 1..24: note = R1 primer for Prkdc
  source 1..24: mol_type = other DNA
gctccagaactcactcttaggctc

SEQ ID NO: 69 - DNA, 20 bp, synthetic construct
  misc_feature 1..20: note = Description of Artificial Sequence: Synthetic oligonucleotide
  misc_feature 1..20: note = Primer for Foxn1
  source 1..20: mol_type = other DNA
ctactccctccgcagtctga

SEQ ID NO: 70 - DNA, 20 bp, synthetic construct
  misc_feature 1..20: note = Description of Artificial Sequence: Synthetic oligonucleotide
  misc_feature 1..20: note = Primer for Foxn1
  source 1..20: mol_type = other DNA
ccaggcctaggttccaggta

SEQ ID NO: 71 - DNA, 20 bp, synthetic construct
  misc_feature 1..20: note = Description of Artificial Sequence: Synthetic oligonucleotide
  misc_feature 1..20: note = Primer for Prkdc
  source 1..20: mol_type = other DNA
ccccagcattgcagatttcc

SEQ ID NO: 72 - DNA, 23 bp, synthetic construct
  misc_feature 1..23: note = Description of Artificial Sequence: Synthetic oligonucleotide
  misc_feature 1..23: note = Primer for Prkdc
  source 1..23: mol_type = other DNA
agggcttcttctctacaatcacg

SEQ ID NO: 73 - DNA, 86 bp, synthetic construct
  misc_feature 1..86: note = Description of Artificial Sequence: Synthetic oligonucleotide
  misc_feature 1..86: note = BRI1 target 1
  source 1..86: mol_type = other DNA
gaaattaatacgactcactataggtttgaaagatggaagcgcgggttttagagctagaaatagcaagttaaaataaggctagtccg

SEQ ID NO: 74 - DNA, 86 bp, synthetic construct
  misc_feature 1..86: note = Description of Artificial Sequence: Synthetic oligonucleotide
  misc_feature 1..86: note = BRI1 target 2
  source 1..86: mol_type = other DNA
gaaattaatacgactcactataggtgaaactaaactggtccacagttttagagctagaaatagcaagttaaaataaggctagtccg

SEQ ID NO: 75 - DNA, 64 bp, synthetic construct
  misc_feature 1..64: note = Description of Artificial Sequence: Synthetic oligonucleotide
  misc_feature 1..64: note = Universal
  source 1..64: mol_type = other DNA
aaaaaagcaccgactcggtgccactttttcaagttgataacggactagccttattttaacttgc

SEQ ID NO: 76 - DNA, 65 bp, synthetic construct
  misc_feature 1..65: note = Description of Artificial Sequence: Synthetic oligonucleotide
  misc_feature 1..65: note = Templates for crRNA
  modified_base 25..44: mod_base = OTHER; note = a, c, t, g, or unknown
  source 1..65: mol_type = other DNA
gaaattaatacgactcactataggnnnnnnnnnnnnnnnnnnnngttttagagctatgctgtttt

SEQ ID NO: 77 - DNA, 67 bp, synthetic construct
  misc_feature 1..67: note = Description of Artificial Sequence: Synthetic oligonucleotide
  misc_feature 1..67: note = tracrRNA
  source 1..67: mol_type = other DNA
gaaattaatacgactcactataggaaccattcaaaacagcatagcaagttaaaataaggctagtccg

SEQ ID NO: 78 - DNA, 69 bp, synthetic construct
  misc_feature 1..69: note = Description of Artificial Sequence: Synthetic oligonucleotide
  misc_feature 1..69: note = tracrRNA
  source 1..69: mol_type = other DNA
aaaaaaagcaccgactcggtgccactttttcaagttgataacggactagccttattttaacttgctatg

SEQ ID NO: 79 - DNA, 20 bp, synthetic construct
  misc_feature 1..20: note = Description of Artificial Sequence: Synthetic oligonucleotide
  misc_feature 1..20: note = Primer
  source 1..20: mol_type = other DNA
ctccatggtgctatagagca

SEQ ID NO: 80 - DNA, 21 bp, synthetic construct
  misc_feature 1..21: note = Description of Artificial Sequence: Synthetic oligonucleotide
  misc_feature 1..21: note = Primer
  source 1..21: mol_type = other DNA
gagccaagctctccatctagt

SEQ ID NO: 81 - DNA, 20 bp, synthetic construct
  misc_feature 1..20: note = Description of Artificial Sequence: Synthetic oligonucleotide
  misc_feature 1..20: note = Primer
  source 1..20: mol_type = other DNA
gccctgtcaagagttgacac

SEQ ID NO: 82 - DNA, 22 bp, synthetic construct
  misc_feature 1..22: note = Description of Artificial Sequence: Synthetic oligonucleotide
  misc_feature 1..22: note = Primer
  source 1..22: mol_type = other DNA
gcacagggtggaacaagatgga

SEQ ID NO: 83 - DNA, 24 bp, synthetic construct
  misc_feature 1..24: note = Description of Artificial Sequence: Synthetic oligonucleotide
  misc_feature 1..24: note = Primer
  source 1..24: mol_type = other DNA
gccaggtacctatcgattgtcagg

SEQ ID NO: 84 - DNA, 21 bp, synthetic construct
  misc_feature 1..21: note = Description of Artificial Sequence: Synthetic oligonucleotide
  misc_feature 1..21: note = Primer
  source 1..21: mol_type = other DNA
gagccaagctctccatctagt

SEQ ID NO: 85 - DNA, 20 bp, synthetic construct
  misc_feature 1..20: note = Description of Artificial Sequence: Synthetic oligonucleotide
  misc_feature 1..20: note = Primer
  source 1..20: mol_type = other DNA
actctgactgggtcaccagc

SEQ ID NO: 86 - DNA, 20 bp, synthetic construct
  misc_feature 1..20: note = Description of Artificial Sequence: Synthetic oligonucleotide
  misc_feature 1..20: note = Primer
  source 1..20: mol_type = other DNA
tatttggctggttgaaaggg

SEQ ID NO: 87 - DNA, 24 bp, synthetic construct
  misc_feature 1..24: note = Description of Artificial Sequence: Synthetic oligonucleotide
  misc_feature 1..24: note = Primer
  source 1..24: mol_type = other DNA
aaagtcatgaaataaacacaccca

SEQ ID NO: 88 - DNA, 24 bp, synthetic construct
  misc_feature 1..24: note = Description of Artificial Sequence: Synthetic oligonucleotide
  misc_feature 1..24: note = Primer
  source 1..24: mol_type = other DNA
ctgcattgatatggtagtaccatg

SEQ ID NO: 89 - DNA, 21 bp, synthetic construct
  misc_feature 1..21: note = Description of Artificial Sequence: Synthetic oligonucleotide
  misc_feature 1..21: note = Primer
  source 1..21: mol_type = other DNA
gctgttcattgcaatggaatg

SEQ ID NO: 90 - DNA, 22 bp, synthetic construct
  misc_feature 1..22: note = Description of Artificial Sequence: Synthetic oligonucleotide
  misc_feature 1..22: note = Primer
  source 1..22: mol_type = other DNA
atggagttggacatggccatgg

SEQ ID NO: 91 - DNA, 28 bp, synthetic construct
  misc_feature 1..28: note = Description of Artificial Sequence: Synthetic oligonucleotide
  misc_feature 1..28: note = Primer
  source 1..28: mol_type = other DNA
actcactatccacagttcagcatttacc

SEQ ID NO: 92 - DNA, 23 bp, synthetic construct
  misc_feature 1..23: note = Description of Artificial Sequence: Synthetic oligonucleotide
  misc_feature 1..23: note = Primer
  source 1..23: mol_type = other DNA
tggagatagctgtcagcaacttt

SEQ ID NO: 93 - DNA, 29 bp, synthetic construct
  misc_feature 1..29: note = Description of Artificial Sequence: Synthetic oligonucleotide
  misc_feature 1..29: note = Primer
  source 1..29: mol_type = other DNA
caacaaagcaaaggtaaagttggtaatag

SEQ ID NO: 94 - DNA, 25 bp, synthetic construct
  misc_feature 1..25: note = Description of Artificial Sequence: Synthetic oligonucleotide
  misc_feature 1..25: note = Primer
  source 1..25: mol_type = other DNA
ggtttcaggagatgtgttacaaggc

SEQ ID NO: 95 - DNA, 27 bp, synthetic construct
  misc_feature 1..27: note = Description of Artificial Sequence: Synthetic oligonucleotide
  misc_feature 1..27: note = Primer
  source 1..27: mol_type = other DNA
gattgtgcaattcctatgcaatcggtc

SEQ ID NO: 96 - DNA, 25 bp, synthetic construct
  misc_feature 1..25: note = Description of Artificial Sequence: Synthetic oligonucleotide
  misc_feature 1..25: note = Primer
  source 1..25: mol_type = other DNA
cactgggtacttaatctgtagcctc

SEQ ID NO: 97 - DNA, 23 bp, synthetic construct
  misc_feature 1..23: note = Description of Artificial Sequence: Synthetic oligonucleotide
  misc_feature 1..23: note = Primer
  source 1..23: mol_type = other DNA
ggttccaagtcattcccagtagc

SEQ ID NO: 98 - DNA, 30 bp, synthetic construct
  misc_feature 1..30: note = Description of Artificial Sequence: Synthetic oligonucleotide
  misc_feature 1..30: note = Primer
  source 1..30: mol_type = other DNA
catcactgcagttgtaggttataactatcc

SEQ ID NO: 99 - DNA, 26 bp, synthetic construct
  misc_feature 1..26: note = Description of Artificial Sequence: Synthetic oligonucleotide
  misc_feature 1..26: note = Primer
  source 1..26: mol_type = other DNA
ttgaaaaccacagatctggttgaacc

SEQ ID NO: 100 - DNA, 22 bp, synthetic construct
  misc_feature 1..22: note = Description of Artificial Sequence: Synthetic oligonucleotide
  misc_feature 1..22: note = Primer
  source 1..22: mol_type = other DNA
ggagtgccaagagaatatctgg

SEQ ID NO: 101 - DNA, 32 bp, synthetic construct
  misc_feature 1..32: note = Description of Artificial Sequence: Synthetic oligonucleotide
  misc_feature 1..32: note = Primer
  source 1..32: mol_type = other DNA
ctgaaactggtttcaaaatattcgttttaagg

SEQ ID NO: 102 - DNA, 22 bp, synthetic construct
  misc_feature 1..22: note = Description of Artificial Sequence: Synthetic oligonucleotide
  misc_feature 1..22: note = Primer
  source 1..22: mol_type = other DNA
gctctgtatgccctgtagtagg

SEQ ID NO: 103 - DNA, 22 bp, synthetic construct
  misc_feature 1..22: note = Description of Artificial Sequence: Synthetic oligonucleotide
  misc_feature 1..22: note = Primer
  source 1..22: mol_type = other DNA
tttgcatctgaccttacctttg

SEQ ID NO: 104 - DNA, 23 bp, synthetic construct
  misc_feature 1..23: note = Description of Artificial Sequence: Synthetic oligonucleotide
  misc_feature 1..23: note = Target sequence of RGEN
  source 1..23: mol_type = other DNA
aatgaccactacatcctcaaggg

SEQ ID NO: 105 - DNA, 23 bp, synthetic construct
  misc_feature 1..23: note = Description of Artificial Sequence: Synthetic oligonucleotide
  misc_feature 1..23: note = Target sequence of RGEN
  source 1..23: mol_type = other DNA
agatgatgtctcatcatcagagg

SEQ ID NO: 106 - DNA, 4170 bp, synthetic construct
  misc_feature 1..4170: note = Description of Artificial Sequence: Synthetic polynucleotide
  misc_feature 1..4170: note = Cas9-coding sequence in p3s-Cas9HC (humanized, C-term tagging, human cell experiments)
  source 1..4170: mol_type = other DNA
atggacaagaagtacagcatcggcctggacatcggtaccaacagcgtgggctgggccgtgatcaccgacgagtacaaggtgcccagcaagaagttcaaggtgctgggcaacaccgaccgccacagcatcaagaagaacctgatcggcgccctgctgttcgacagcggcgagaccgccgaggccacccgcctgaagcgcaccgcccgccgccgctacacccgccgcaagaaccgcatctgctacctgcaggagatcttcagcaacgagatggccaaggtggacgacagcttcttccaccgcctggaggagagcttcctggtggaggaggacaagaagcacgagcgccaccccatcttcggcaacatcgtggacgaggtggcctaccacgagaagtaccccaccatctaccacctgcgcaagaagctggtggacagcaccgacaaggccgacctgcgcctgatctacctggccctggcccacatgatcaagttccgcggccacttcctgatcgagggcgacctgaaccccgacaacagcgacgtggacaagctgttcatccagctggtgcagacctacaaccagctgttcgaggagaaccccatcaacgccagcggcgtggacgccaaggccatcctgagcgcccgcctgagcaagagccgccgcctggagaacctgatcgcccagctgcccggcgagaagaagaacggcctgttcggcaacctgatcgccctgagcctgggcctgacccccaacttcaagagcaacttcgacctggccgaggacgccaagctgcagctgagcaaggacacctacgacgacgacctggacaacctgctggcccagatcggcgaccagtacgccgacctgttcctggccgccaagaacctgagcgacgccatcctgctgagcgacatcctgcgcgtgaacaccgagatcaccaaggcccccctgagcgccagcatgatcaagcgctacgacgagcaccaccaggacctgaccctgctgaaggccctggtgcgccagcagctgcccgagaagtacaaggagatcttcttcgaccagagcaagaacggctacgccggctacatcgacggcggcgccagccaggaggagttctacaagttcatcaagcccatcctggagaagatggacggcaccgaggagctgctggtgaagctgaaccgcgaggacctgctgcgcaagcagcgcaccttcgacaacggcagcatcccccaccagatccacctgggcgagctgcacgccatcctgcgccgccaggaggacttctaccccttcctgaaggacaaccgcgagaagatcgagaagatcctgaccttccgcatcccctactacgtgggccccctggcccgcggcaacagccgcttcgcctggatgacccgcaagagcgaggagaccatcaccccctggaacttcgaggaggtggtggacaagggcgccagcgcccagagcttcatcgagcgcatgaccaacttcgacaagaacctgcccaacgagaaggtgctgcccaagcacagcctgctgtacgagtacttcaccgtgtacaacgagctgaccaaggtgaagtacgtgaccgagggcatgcgcaagcccgccttcctgagcggcgagcagaagaaggccatcgtggacctgctgttcaagaccaaccgcaaggtgaccgtgaagcagctgaaggaggactacttcaagaagatcgagtgcttcgacagcgtggagatcagcggcgtggaggaccgcttcaacgccagcctgggcacctaccacgacctgctgaagatcatcaaggacaaggacttcctggacaacgaggagaacgaggacatcctggaggacatcgtgctgaccctgaccctgttcgaggaccgcgagatgatcgaggagcgcctgaagacctacgcccacctgttcgacgacaaggtgatgaagcagctgaagcgccgccgctacaccggctggggccgcctgagccgcaagcttatcaacggcatccgcgacaagcagagcggcaagaccatcctggacttcctgaagagcgacggcttcgccaaccgcaacttcatgcagctgatccacgacgacagcctgaccttcaaggaggacatccagaaggcccaggtgagcggccagggcgacagcctgcacgagcacatcgccaacctggccggcagccccgccatcaagaagggcatcctgcagaccgtgaaggtggtggacgagctggtgaaggtgatgggccgccacaagcccgagaacatcgtgatcgagatggcccgcgagaaccagaccacccagaagggccagaagaacagccgcgagcgcatgaagcgcatcgaggagggcatcaaggagctgggcagccagatcctgaaggagcaccccgtggagaacacccagctgcagaacgagaagctgtacctgtactacctgcagaacggccgcgacatgtacgtggaccaggagctggacatcaaccgcctgagcgactacgacgtggaccacatcgtgccccagagcttcctgaaggacgacagcatcgacaacaaggtgctgacccgcagcgacaagaaccgcggcaagagcgacaacgtgcccagcgaggaggtggtgaagaagatgaagaactactggcgccagctgctgaacgccaagctgatcacccagcgcaagttcgacaacctgaccaaggccgagcgcggcggcctgagcgagctggacaaggccggcttcatcaagcgccagctggtggagacccgccagatcaccaagcacgtggcccagatcctggacagccgcatgaacaccaagtacgacgagaacgacaagctgatccgcgaggtgaaggtgatcaccctgaagagcaagctggtgagcgacttccgcaaggacttccagttctacaaggtgcgcgagatcaacaactaccaccacgcccacgacgcctacctgaacgccgtggtgggcaccgccctgatcaagaagtaccccaagctggagagcgagttcgtgtacggcgactacaaggtgtacgacgtgcgcaagatgatcgccaagagcgagcaggagatcggcaaggccaccgccaagtacttcttctacagcaacatcatgaacttcttcaagaccgagatcaccctggccaacggcgagatccgcaagcgccccctgatcgagaccaacggcgagaccggcgagatcgtgtgggacaagggccgcgacttcgccaccgtgcgcaaggtgctgagcatgccccaggtgaacatcgtgaagaagaccgaggtgcagaccggcggcttcagcaaggagagcatcctgcccaagcgcaacagcgacaagctgatcgcccgcaagaaggactgggaccccaagaagtacggcggcttcgacagccccaccgtggcctacagcgtgctggtggtggccaaggtggagaagggcaagagcaagaagctgaagagcgtgaaggagctgctgggcatcaccatcatggagcgcagcagcttcgagaagaaccccatcgacttcctggaggccaagggctacaaggaggtgaagaaggacctgatcatcaagctgcccaagtacagcctgttcgagctggagaacggccgcaagcgcatgctggccagcgccggcgagctgcagaagggcaacgagctggccctgcccagcaagtacgtgaacttcctgtacctggccagccactacgagaagctgaagggcagccccgaggacaacgagcagaagcagctgttcgtggagcagcacaagcactacctggacgagatcatcgagcagatcagcgagttcagcaagcgcgtgatcctggccgacgccaacctggacaaggtgctgagcgcctacaacaagcaccgcgacaagcccatccgcgagcaggccgagaacatcatccacctgttcaccctgaccaacctgggcgcccccgccgccttcaagtacttcgacaccaccatcgaccgcaagcgctacaccagcaccaaggaggtgctggacgccaccctgatccaccagagcatcaccggtctgtacgagacccgcatcgacctgagccagctgggcggcgacggcggctccggacctccaaagaaaaagagaaaagtatacccctacgacgtgcccgactacgcctaa

SEQ ID NO: 107 - DNA, 4194 bp, synthetic construct
  misc_feature 1..4194: note = Description of Artificial Sequence: Synthetic polynucleotide
  misc_feature 1..4194: note = Cas9 coding sequence in p3s-Cas9HN (humanized codon, N-term tagging (underlined), human cell experiments)
  source 1..4194: mol_type = other DNA
atggtgtacccctacgacgtgcccgactacgccgaattgcctccaaaaaagaagagaaaggtagggatccgaattcccggggaaaaaccggacaagaagtacagcatcggcctggacatcggtaccaacagcgtgggctgggccgtgatcaccgacgagtacaaggtgcccagcaagaagttcaaggtgctgggcaacaccgaccgccacagcatcaagaagaacctgatcggcgccctgctgttcgacagcggcgagaccgccgaggccacccgcctgaagcgcaccgcccgccgccgctacacccgccgcaagaaccgcatctgctacctgcaggagatcttcagcaacgagatggccaaggtggacgacagcttcttccaccgcctggaggagagcttcctggtggaggaggacaagaagcacgagcgccaccccatcttcggcaacatcgtggacgaggtggcctaccacgagaagtaccccaccatctaccacctgcgcaagaagctggtggacagcaccgacaaggccgacctgcgcctgatctacctggccctggcccacatgatcaagttccgcggccacttcctgatcgagggcgacctgaaccccgacaacagcgacgtggacaagctgttcatccagctggtgcagacctacaaccagctgttcgaggagaaccccatcaacgccagcggcgtggacgccaaggccatcctgagcgcccgcctgagcaagagccgccgcctggagaacctgatcgcccagctgcccggcgagaagaagaacggcctgttcggcaacctgatcgccctgagcctgggcctgacccccaacttcaagagcaacttcgacctggccgaggacgccaagctgcagctgagcaaggacacctacgacgacgacctggacaacctgctggcccagatcggcgaccagtacgccgacctgttcctggccgccaagaacctgagcgacgccatcctgctgagcgacatcctgcgcgtgaacaccgagatcaccaaggcccccctgagcgccagcatgatcaagcgctacgacgagcaccaccaggacctgaccctgctgaaggccctggtgcgccagcagctgcccgagaagtacaaggagatcttcttcgaccagagcaagaacggctacgccggctacatcgacggcggcgccagccaggaggagttctacaagttcatcaagcccatcctggagaagatggacggcaccgaggagctgctggtgaagctgaaccgcgaggacctgctgcgcaagcagcgcaccttcgacaacggcagcatcccccaccagatccacctgggcgagctgcacgccatcctgcgccgccaggaggacttctaccccttcctgaaggacaaccgcgagaagatcgagaagatcctgaccttccgcatcccctactacgtgggccccctggcccgcggcaacagccgcttcgcctggatgacccgcaagagcgaggagaccatcaccccctggaacttcgaggaggtggtggacaagggcgccagcgcccagagcttcatcgagcgcatgaccaacttcgacaagaacctgcccaacgagaaggtgctgcccaagcacagcctgctgtacgagtacttcaccgtgtacaacgagctgaccaaggtgaagtacgtgaccgagggcatgcgcaagcccgccttcctgagcggcgagcagaagaaggccatcgtggacctgctgttcaagaccaaccgcaaggtgaccgtgaagcagctgaaggaggactacttcaagaagatcgagtgcttcgacagcgtggagatcagcggcgtggaggaccgcttcaacgccagcctgggcacctaccacgacctgctgaagatcatcaaggacaaggacttcctggacaacgaggagaacgaggacatcctggaggacatcgtgctgaccctgaccctgttcgaggaccgcgagatgatcgaggagcgcctgaagacctacgcccacctgttcgacgacaaggtgatgaagcagctgaagcgccgccgctacaccggctggggccgcctgagccgcaagcttatcaacggcatccgcgacaagcagagcggcaagaccatcctggacttcctgaagagcgacggcttcgccaaccgcaacttcatgcagctgatccacgacgacagcctgaccttcaaggaggacatccagaaggcccaggtgagcggccagggcgacagcctgcacgagcacatcgccaacctggccggcagccccgccatcaagaagggcatcctgcagaccgtgaaggtggtggacgagctggtgaaggtgatgggccgccacaagcccgagaacatcgtgatcgagatggcccgcgagaaccagaccacccagaagggccagaagaacagccgcgagcgcatgaagcgcatcgaggagggcatcaaggagctgggcagccagatcctgaaggagcaccccgtggagaacacccagctgcagaacgagaagctgtacctgtactacctgcagaacggccgcgacatgtacgtggaccaggagctggacatcaaccgcctgagcgactacgacgtggaccacatcgtgccccagagcttcctgaaggacgacagcatcgacaacaaggtgctgacccgcagcgacaagaaccgcggcaagagcgacaacgtgcccagcgaggaggtggtgaagaagatgaagaactactggcgccagctgctgaacgccaagctgatcacccagcgcaagttcgacaacctgaccaaggccgagcgcggcggcctgagcgagctggacaaggccggcttcatcaagcgccagctggtggagacccgccagatcaccaagcacgtggcccagatcctggacagccgcatgaacaccaagtacgacgagaacgacaagctgatccgcgaggtgaaggtgatcaccctgaagagcaagctggtgagcgacttccgcaaggacttccagttctacaaggtgcgcgagatcaacaactaccaccacgcccacgacgcctacctgaacgccgtggtgggcaccgccctgatcaagaagtaccccaagctggagagcgagttcgtgtacggcgactacaaggtgtacgacgtgcgcaagatgatcgccaagagcgagcaggagatcggcaaggccaccgccaagtacttcttctacagcaacatcatgaacttcttcaagaccgagatcaccctggccaacggcgagatccgcaagcgccccctgatcgagaccaacggcgagaccggcgagatcgtgtgggacaagggccgcgacttcgccaccgtgcgcaaggtgctgagcatgccccaggtgaacatcgtgaagaagaccgaggtgcagaccggcggcttcagcaaggagagcatcctgcccaagcgcaacagcgacaagctgatcgcccgcaagaaggactgggaccccaagaagtacggcggcttcgacagccccaccgtggcctacagcgtgctggtggtggccaaggtggagaagggcaagagcaagaagctgaagagcgtgaaggagctgctgggcatcaccatcatggagcgcagcagcttcgagaagaaccccatcgacttcctggaggccaagggctacaaggaggtgaagaaggacctgatcatcaagctgcccaagtacagcctgttcgagctggagaacggccgcaagcgcatgctggccagcgccggcgagctgcagaagggcaacgagctggccctgcccagcaagtacgtgaacttcctgtacctggccagccactacgagaagctgaagggcagccccgaggacaacgagcagaagcagctgttcgtggagcagcacaagcactacctggacgagatcatcgagcagatcagcgagttcagcaagcgcgtgatcctggccgacgccaacctggacaaggtgctgagcgcctacaacaagcaccgcgacaagcccatccgcgagcaggccgagaacatcatccacctgttcaccctgaccaacctgggcgcccccgccgccttcaagtacttcgacaccaccatcgaccgcaagcgctacaccagcaccaaggaggtgctggacgccaccctgatccaccagagcatcaccggtctgtacgagacccgcatcgacctgagccagctgggcggcgactaa

SEQ ID NO: 108 - DNA, 4107 bp, synthetic construct
  misc_feature 1..4107: note = Description of Artificial Sequence: Synthetic polynucleotide
  misc_feature 1..4107: note = Cas9-coding sequence in Streptococcus pyogenes
  source 1..4107: mol_type = other DNA
atggataagaaatactcaataggcttagatatcggcacaaatagcgtcggatgggcggtgatcactgatgaatataaggttccgtctaaaaagttcaaggttctgggaaatacagaccgccacagtatcaaaaaaaatcttataggggctcttttatttgacagtggagagacagcggaagcgactcgtctcaaacggacagctcgtagaaggtatacacgtcggaagaatcgtatttgttatctacaggagattttttcaaatgagatggcgaaagtagatgatagtttctttcatcgacttgaagagtcttttttggtggaagaagacaagaagcatgaacgtcatcctatttttggaaatatagtagatgaagttgcttatcatgagaaatatccaactatctatcatctgcgaaaaaaattggtagattctactgataaagcggatttgcgcttaatctatttggccttagcgcatatgattaagtttcgtggtcattttttgattgagggagatttaaatcctgataatagtgatgtggacaaactatttatccagttggtacaaacctacaatcaattatttgaagaaaaccctattaacgcaagtggagtagatgctaaagcgattctttctgcacgattgagtaaatcaagacgattagaaaatctcattgctcagctccccggtgagaagaaaaatggcttatttgggaatctcattgctttgtcattgggtttgacccctaattttaaatcaaattttgatttggcagaagatgctaaattacagctttcaaaagatacttacgatgatgatttagataatttattggcgcaaattggagatcaatatgctgatttgtttttggcagctaagaatttatcagatgctattttactttcagatatcctaagagtaaatactgaaataactaaggctcccctatcagcttcaatgattaaacgctacgatgaacatcatcaagacttgactcttttaaaagctttagttcgacaacaacttccagaaaagtataaagaaatcttttttgatcaatcaaaaaacggatatgcaggttatattgatgggggagctagccaagaagaattttataaatttatcaaaccaattttagaaaaaatggatggtactgaggaattattggtgaaactaaatcgtgaagatttgctgcgcaagcaacggacctttgacaacggctctattccccatcaaattcacttgggtgagctgcatgctattttgagaagacaagaagacttttatccatttttaaaagacaatcgtgagaagattgaaaaaatcttgacttttcgaattccttattatgttggtccattggcgcgtggcaatagtcgttttgcatggatgactcggaagtctgaagaaacaattaccccatggaattttgaagaagttgtcgataaaggtgcttcagctcaatcatttattgaacgcatgacaaactttgataaaaatcttccaaatgaaaaagtactaccaaaacatagtttgctttatgagtattttacggtttataacgaattgacaaaggtcaaatatgttactgaaggaatgcgaaaaccagcatttctttcaggtgaacagaagaaagccattgttgatttactcttcaaaacaaatcgaaaagtaaccgttaagcaattaaaagaagattatttcaaaaaaatagaatgttttgatagtgttgaaatttcaggagttgaagatagatttaatgcttcattaggtacctaccatgatttgctaaaaattattaaagataaagattttttggataatgaagaaaatgaagatatcttagaggatattgttttaacattgaccttatttgaagatagggagatgattgaggaaagacttaaaacatatgctcacctctttgatgataaggtgatgaaacagcttaaacgtcgccgttatactggttggggacgtttgtctcgaaaattgattaatggtattagggataagcaatctggcaaaacaatattagattttttgaaatcagatggttttgccaatcgcaattttatgcagctgatccatgatgatagtttgacatttaaagaagacattcaaaaagcacaagtgtctggacaaggcgatagtttacatgaacatattgcaaatttagctggtagccctgctattaaaaaaggtattttacagactgtaaaagttgttgatgaattggtcaaagtaatggggcggcataagccagaaaatatcgttattgaaatggcacgtgaaaatcagacaactcaaaagggccagaaaaattcgcgagagcgtatgaaacgaatcgaagaaggtatcaaagaattaggaagtcagattcttaaagagcatcctgttgaaaatactcaattgcaaaatgaaaagctctatctctattatctccaaaatggaagagacatgtatgtggaccaagaattagatattaatcgtttaagtgattatgatgtcgatcacattgttccacaaagtttccttaaagacgattcaatagacaataaggtcttaacgcgttctgataaaaatcgtggtaaatcggataacgttccaagtgaagaagtagtcaaaaagatgaaaaactattggagacaacttctaaacgccaagttaatcactcaacgtaagtttgataatttaacgaaagctgaacgtggaggtttgagtgaacttgataaagctggttttatcaaacgccaattggttgaaactcgccaaatcactaagcatgtggcacaaattttggatagtcgcatgaatactaaatacgatgaaaatgataaacttattcgagaggttaaagtgattaccttaaaatctaaattagtttctgacttccgaaaagatttccaattctataaagtacgtgagattaacaattaccatcatgcccatgatgcgtatctaaatgccgtcgttggaactgctttgattaagaaatatccaaaacttgaatcggagtttgtctatggtgattataaagtttatgatgttcgtaaaatgattgctaagtctgagcaagaaataggcaaagcaaccgcaaaatatttcttttactctaatatcatgaacttcttcaaaacagaaattacacttgcaaatggagagattcgcaaacgccctctaatcgaaactaatggggaaactggagaaattgtctgggataaagggcgagattttgccacagtgcgcaaagtattgtccatgccccaagtcaatattgtcaagaaaacagaagtacagacaggcggattctccaaggagtcaattttaccaaaaagaaattcggacaagcttattgctcgtaaaaaagactgggatccaaaaaaatatggtggttttgatagtccaacggtagcttattcagtcctagtggttgctaaggtggaaaaagggaaatcgaagaagttaaaatccgttaaagagttactagggatcacaattatggaaagaagttcctttgaaaaaaatccgattgactttttagaagctaaaggatataaggaagttaaaaaagacttaatcattaaactacctaaatatagtctttttgagttagaaaacggtcgtaaacggatgctggctagtgccggagaattacaaaaaggaaatgagctggctctgccaagcaaatatgtgaattttttatatttagctagtcattatgaaaagttgaagggtagtccagaagataacgaacaaaaacaattgtttgtggagcagcataagcattatttagatgagattattgagcaaatcagtgaattttctaagcgtgttattttagcagatgccaatttagataaagttcttagtgcatataacaaacatagagacaaaccaatacgtgaacaagcagaaaatattattcatttatttacgttgacgaatcttggagctcccgctgcttttaaatattttgatacaacaattgatcgtaaacgatatacgtctacaaaagaagttttagatgccactcttatccatcaatccatcactggtctttatgaaacacgcattgatttgagtcagctaggaggtgactaa

SEQ ID NO: 109 - protein, 1368 aa, synthetic construct [sequence omitted]

SEQ ID NO: 110 - DNA, 4221 bp, synthetic construct
  misc_feature 1..4221: note = Description of Artificial Sequence: Synthetic polynucleotide
  misc_feature 1..4221: note = Cas9-coding sequence in pET-Cas9N3T for the production of recombinant Cas9 protein in E. coli (humanized codon; hexa-His-tag and a nuclear localization signal at the N terminus)
  source 1..4221: mol_type = other DNA
atgggcagcagccatcatcatcatcatcatgtgtacccctacgacgtgcccgactacgccgaattgcctccaaaaaagaagagaaaggtagggatcgagaacctgtacttccagggcgacaagaagtacagcatcggcctggacatcggtaccaacagcgtgggctgggccgtgatcaccgacgagtacaaggtgcccagcaagaagttcaaggtgctgggcaacaccgaccgccacagcatcaagaagaacctgatcggcgccctgctgttcgacagcggcgagaccgccgaggccacccgcctgaagcgcaccgcccgccgccgctacacccgccgcaagaaccgcatctgctacctgcaggagatcttcagcaacgagatggccaaggtggacgacagcttcttccaccgcctggaggagagcttcctggtggaggaggacaagaagcacgagcgccaccccatcttcggcaacatcgtggacgaggtggcctaccacgagaagtaccccaccatctaccacctgcgcaagaagctggtggacagcaccgacaaggccgacctgcgcctgatctacctggccctggcccacatgatcaagttccgcggccacttcctgatcgagggcgacctgaaccccgacaacagcgacgtggacaagctgttcatccagctggtgcagacctacaaccagctgttcgaggagaaccccatcaacgccagcggcgtggacgccaaggccatcctgagcgcccgcctgagcaagagccgccgcctggagaacctgatcgcccagctgcccggcgagaagaagaacggcctgttcggcaacctgatcgccctgagcctgggcctgacccccaacttcaagagcaacttcgacctggccgaggacgccaagctgcagctgagcaaggacacctacgacgacgacctggacaacctgctggcccagatcggcgaccagtacgccgacctgttcctggccgccaagaacctgagcgacgccatcctgctgagcgacatcctgcgcgtgaacaccgagatcaccaaggcccccctgagcgccagcatgatcaagcgctacgacgagcaccaccaggacctgaccctgctgaaggccctggtgcgccagcagctgcccgagaagtacaaggagatcttcttcgaccagagcaagaacggctacgccggctacatcgacggcggcgccagccaggaggagttctacaagttcatcaagcccatcctggagaagatggacggcaccgaggagctgctggtgaagctgaaccgcgaggacctgctgcgcaagcagcgcaccttcgacaacggcagcatcccccaccagatccacctgggcgagctgcacgccatcctgcgccgccaggaggacttctaccccttcctgaaggacaaccgcgagaagatcgagaagatcctgaccttccgcatcccctactacgtgggccccctggcccgcggcaacagccgcttcgcctggatgacccgcaagagcgaggagaccatcaccccctggaacttcgaggaggtggtggacaagggcgccagcgcccagagcttcatcgagcgcatgaccaacttcgacaagaacctgcccaacgagaaggtgctgcccaagcacagcctgctgtacgagtacttcaccgtgtacaacgagctgaccaaggtgaagtacgtgaccgagggcatgcgcaagcccgccttcctgagcggcgagcagaagaaggccatcgtggacctgctgttcaagaccaaccgcaaggtgaccgtgaagcagctgaaggaggactacttcaagaagatcgagtgcttcgacagcgtggagatcagcggcgtggaggaccgcttcaacgccagcctgggcacctaccacgacctgctgaagatcatcaaggacaaggacttcctggacaacgaggagaacgaggacatcctggaggacatcgtgctgaccctgaccctgttcgaggaccgcgagatgatcgaggagcgcctgaagacctacgcccacctgttcgacgacaaggtgatgaagcagctgaagcgccgccgctacaccggctggggccgcctgagccgcaagcttatcaacggcatccgcgacaagcagagcggcaagaccatcctggacttcctgaagagcgacggcttcgccaaccgcaacttcatgcagctgatccacgacgacagcctgaccttcaaggaggacatccagaaggcccaggtgagcggccagggcgacagcctgcacgagcacatcgccaacctggccggcagccccgccatcaagaagggcatcctgcagaccgtgaaggtggtggacgagctggtgaaggtgatgggccgccacaagcccgagaacatcgtgatcgagatggcccgcgagaaccagaccacccagaagggccagaagaacagccgcgagcgcatgaagcgcatcgaggagggcatcaaggagctgggcagccagatcctgaaggagcaccccgtggagaacacccagctgcagaacgagaagctgtacctgtactacctgcagaacggccgcgacatgtacgtggaccaggagctggacatcaaccgcctgagcgactacgacgtggaccacatcgtgccccagagcttcctgaaggacgacagcatcgacaacaaggtgctgacccgcagcgacaagaaccgcggcaagagcgacaacgtgcccagcgaggaggtggtgaagaagatgaagaactactggcgccagctgctgaacgccaagctgatcacccagcgcaagttcgacaacctgaccaaggccgagcgcggcggcctgagcgagctggacaaggccggcttcatcaagcgccagctggtggagacccgccagatcaccaagcacgtggcccagatcctggacagccgcatgaacaccaagtacgacgagaacgacaagctgatccgcgaggtgaaggtgatcaccctgaagagcaagctggtgagcgacttccgcaaggacttccagttctacaaggtgcgcgagatcaacaactaccaccacgcccacgacgcctacctgaacgccgtggtgggcaccgccctgatcaagaagtaccccaagctggagagcgagttcgtgtacggcgactacaaggtgtacgacgtgcgcaagatgatcgccaagagcgagcaggagatcggcaaggccaccgccaagtacttcttctacagcaacatcatgaacttcttcaagaccgagatcaccctggccaacggcgagatccgcaagcgccccctgatcgagaccaacggcgagaccggcgagatcgtgtgggacaagggccgcgacttcgccaccgtgcgcaaggtgctgagcatgccccaggtgaacatcgtgaagaagaccgaggtgcagaccggcggcttcagcaaggagagcatcctgcccaagcgcaacagcgacaagctgatcgcccgcaagaaggactgggaccccaagaagtacggcggcttcgacagccccaccgtggcctacagcgtgctggtggtggccaaggtggagaagggcaagagcaagaagctgaagagcgtgaaggagctgctgggcatcaccatcatggagcgcagcagcttcgagaagaaccccatcgacttcctggaggccaagggctacaaggaggtgaagaaggacctgatcatcaagctgcccaagtacagcctgttcgagctggagaacggccgcaagcgcatgctggccagcgccggcgagctgcagaagggcaacgagctggccctgcccagcaagtacgtgaacttcctgtacctggccagccactacgagaagctgaagggcagccccgaggacaacgagcagaagcagctgttcgtggagcagcacaagcactacctggacgagatcatcgagcagatcagcgagttcagcaagcgcgtgatcctggccgacgccaacctggacaaggtgctgagcgcctacaacaagcaccgcgacaagcccatccgcgagcaggccgagaacatcatccacctgttcaccctgaccaacctgggcgcccccgccgccttcaagtacttcgacaccaccatcgaccgcaagcgctacaccagcaccaaggaggtgctggacgccaccctgatccaccagagcatcaccggtctgtacgagacccgcatcgacctgagccagctgggcggcgactaa

SEQ ID NO: 111 - protein, 1406 aa, synthetic construct
  REGION 1..1406: note = Description of Artificial Sequence: Synthetic polypeptide
  REGION 1..1406: note = Amino acid sequence of Cas9 (pET-Cas9N3T)
MGSSHHHHHHVYPYDVPDYAELPPKKKRKVGIENLYFQGDKKYSIGLDIGTNSVGWAVITDEYKVPSKKFKVLGNTDRHSIKKNLIGALLFDSGETAEATRLKRTARRRYTRRKNRICYLQEIFSNEMAKVDDSFFHRLEESFLVEEDKKHERHPIFGNIVDEVAYHEKYPTIYHLRKKLVDSTDKADLRLIYLALAHMIKFRGHFLIEGDLNPDNSDVDKLFIQLVQTYNQLFEENPINASGVDAKAILSARLSKSRRLENLIAQLPGEKKNGLFGNLIALSLGLTPNFKSNFDLAEDAKLQLSKDTYDDDLDNLLAQIGDQYADLFLAAKNLSDAILLSDILRVNTEITKAPLSASMIKRYDEHHQDLTLLKALVRQQLPEKYKEIFFDQSKNGYAGYIDGGASQEEFYKFIKPILEKMDGTEELLVKLNREDLLRKQRTFDNGSIPHQIHLGELHAILRRQEDFYPFLKDNREKIEKILTFRIPYYVGPLARGNSRFAWMTRKSEETITPWNFEEVVDKGASAQSFIERMTNFDKNLPNEKVLPKHSLLYEYFTVYNELTKVKYVTEGMRKPAFLSGEQKKAIVDLLFKTNRKVTVKQLKEDYFKKIECFDSVEISGVEDRFNASLGTYHDLLKIIKDKDFLDNEENEDILEDIVLTLTLFEDREMIEERLKTYAHLFDDKVMKQLKRRRYTGWGRLSRKLINGIRDKQSGKTILDFLKSDGFANRNFMQLIHDDSLTFKEDIQKAQVSGQGDSLHEHIANLAGSPAIKKGILQTVKVVDELVKVMGRHKPENIVIEMARENQTTQKGQKNSRERMKRIEEGIKELGSQILKEHPVENTQLQNEKLYLYYLQNGRDMYVDQELDINRLSDYDVDHIVPQSFLKDDSIDNKVLTRSDKNRGKSDNVPSEEVVKKMKNYWRQLLNAKLITQRKFDNLTKAERGGLSELDKAGFIKRQLVETRQITKHVAQILDSRMNTKYDENDKLIREVKVITLKSKLVSDFRKDFQFYKVREINNYHHAHDAYLNAVVGTALIKKYPKLESEFVYGDYKVYDVRKMIAKSEQEIGKATAKYFFYSNIMNFFKTEITLANGEIRKRPLIETNGETGEIVWDKGRDFATVRKVLSMPQVNIVKKTEVQTGGFSKESILPKRNSDKLIARKKDWDPKKYGGFDSPTVAYSVLVVAKVEKGKSKKLKSVKELLGITIMERSSFEKNPIDFLEAKGYKEVKKDLIIKLPKYSLFELENGRKRMLASAGELQKGNELALPSKYVNFLYLASHYEKLKGSPEDNEQKQLFVEQHKHYLDEIIEQISEFSKRVILADANLDKVLSAYNKHRDKPIREQAENIIHLFTLTNLGAPAAFKYFDTTIDRKRYTSTKEVLDATLIHQSITGLYETRIDLSQLGGD

SEQ ID NO: 112 - DNA, 34 bp, Homo sapiens
  source 1..34: mol_type = other DNA
caatctatgacatcaattattatacatcggagcc

SEQ ID NO: 113 - RNA, 64 nt, synthetic construct
  misc_feature 1..64: note = Description of Artificial Sequence: Synthetic oligonucleotide
  source 1..64: mol_type = other RNA
ggtgacatcaattattatacatgttttagagctagaaatagcaagttaaaataaggctagtccg

SEQ ID NO: 114 - DNA, 49 bp, synthetic construct
  misc_feature 1..49: note = Description of Artificial Sequence: Synthetic oligonucleotide
  source 1..49: mol_type = other DNA
caatctatgacatcaattattatacatcggagccctgccaaaaaatcaa

SEQ ID NO: 115 - DNA, 50 bp, synthetic construct
  misc_feature 1..50: note = Description of Artificial Sequence: Synthetic oligonucleotide
  source 1..50: mol_type = other DNA
caatctatgacatcaattattataacatcggagccctgccaaaaaatcaa

SEQ ID NO: 116 - DNA, 36 bp, synthetic construct
  misc_feature 1..36: note = Description of Artificial Sequence: Synthetic oligonucleotide
  source 1..36: mol_type = other DNA
caatctatgacatcaattattatgccaaaaaatcaa

SEQ ID NO: 117 - DNA, 35 bp, synthetic construct
  misc_feature 1..35: note = Description of Artificial Sequence: Synthetic oligonucleotide
  source 1..35: mol_type = other DNA
caatctatgacatcggagccctgccaaaaaatcaa

SEQ ID NO: 118 - DNA, 31 bp, synthetic construct
  misc_feature 1..31: note = Description of Artificial Sequence: Synthetic oligonucleotide
  source 1..31: mol_type = other DNA
caatctatgacatgccctgccaaaaaatcaa

SEQ ID NO: 119 - DNA, 30 bp, synthetic construct
  misc_feature 1..30: note = Description of Artificial Sequence: Synthetic oligonucleotide
  source 1..30: mol_type = other DNA
caatctatgacatcaattattataaatcaa

SEQ ID NO: 120 - DNA, 25 bp, synthetic construct
  misc_feature 1..25: note = Description of Artificial Sequence: Synthetic oligonucleotide
  source 1..25: mol_type = other DNA
caatctatgacatccaaaaaatcaa

SEQ ID NO: 121 - DNA, 19 bp, synthetic construct
  misc_feature 1..19: note = Description of Artificial Sequence: Synthetic oligonucleotide
  source 1..19: mol_type = other DNA
caatctatgacaaaatcaa

SEQ ID NO: 122 - DNA, 46 bp, Homo sapiens
  source 1..46: mol_type = other DNA
tatgtgcaatgaccactacatcctcaagggcagcaatcggagccag

SEQ ID NO: 123 - DNA, 47 bp, synthetic construct
  misc_feature 1..47: note = Description of Artificial Sequence: Synthetic oligonucleotide
  source 1..47: mol_type = other DNA
tatgtgcaatgaccactacatccttcaagggcagcaatcggagccag

SEQ ID NO: 124 - DNA, 48 bp, synthetic construct
  misc_feature 1..48: note = Description of Artificial Sequence: Synthetic oligonucleotide
  source 1..48: mol_type = other DNA
tatgtgcaatgaccactacatcctctcaagggcagcaatcggagccag

SEQ ID NO: 125 - DNA, 18 bp, synthetic construct
  misc_feature 1..18: note = Description of Artificial Sequence: Synthetic oligonucleotide
  source 1..18: mol_type = other DNA
tatgtgcaatggagccag

SEQ ID NO: 126 - DNA, 13 bp, synthetic construct
  misc_feature 1..13: note = Description of Artificial Sequence: Synthetic oligonucleotide
  source 1..13: mol_type = other DNA
tatgtgcaatgac

SEQ ID NO: 127 - DNA, 23 bp, Homo sapiens
  source 1..23: mol_type = other DNA
tgacatcaattattatacatcgg

SEQ ID NO: 128 - DNA, 23 bp, Homo sapiens
  source 1..23: mol_type = other DNA
tgacatcaattattatagatgga

SEQ ID NO: 129 - DNA, 23 bp, Homo sapiens
  source 1..23: mol_type = other DNA
tgacatcacttattatgcatggg

SEQ ID NO: 130 - DNA, 23 bp, Homo sapiens
  source 1..23: mol_type = other DNA
tgacataaattattctacatggg

SEQ ID NO: 131 - DNA, 23 bp, Homo sapiens
  source 1..23: mol_type = other DNA
tgaaatcaattatcatagatcgg

SEQ ID NO: 132 - DNA, 23 bp, Homo sapiens
  source 1..23: mol_type = other DNA
ccaggctccacccgactggaggg

SEQ ID NO: 133 - RNA, 106 nt, synthetic construct
  misc_feature 1..106: note = Description of Artificial Sequence: Synthetic polynucleotide
  source 1..106: mol_type = other RNA
ggccaggctccacccgactggagttttagagctagaaatagcaagttaaaataaggctagtccgttatcaacttgaaaaagtggcaccgagtcggtgctttttttt

SEQ ID NO: 134 - DNA, 53 bp, Homo sapiens
  source 1..53: mol_type = other DNA
acttccaggctccacccgactggagggcgaaccccaaggggacctcatgcagg

SEQ ID NO: 135 - DNA, 13 bp, synthetic construct
  misc_feature 1..13: note = Description of Artificial Sequence: Synthetic oligonucleotide
  source 1..13: mol_type = other DNA
acttccaggctcc

SEQ ID NO: 136 - DNA, 30 bp, synthetic construct
  misc_feature 1..30: note = Description of Artificial Sequence: Synthetic oligonucleotide
  source 1..30: mol_type = other DNA
acttccaggctccacccgacctcatgcagg

SEQ ID NO: 137 - DNA, 36 bp, synthetic construct
  misc_feature 1..36: note = Description of Artificial Sequence: Synthetic oligonucleotide
  source 1..36: mol_type = other DNA
acttccaggctccaccccaaggggacctcatgcagg

SEQ ID NO: 138 - DNA, 54 bp, synthetic construct
  misc_feature 1..54: note = Description of Artificial Sequence: Synthetic oligonucleotide
  source 1..54: mol_type = other DNA
acttccaggctccacccgacttggagggcgaaccccaaggggacctcatgcagg

SEQ ID NO: 139 - DNA, 43 bp, synthetic construct
  misc_feature 1..43: note = Description of Artificial Sequence: Synthetic oligonucleotide
  source 1..43: mol_type = other DNA
acttccaggctccacccgaaccccaaggggacctcatgcaggg

SEQ ID NO: 140 - DNA, 47 bp, synthetic construct
  misc_feature 1..47: note = Description of Artificial Sequence: Synthetic oligonucleotide
  source 1..47: mol_type = other DNA
acttccaggctccacccgactcactatcttctgggctcctccatgtc

SEQ ID NO: 141 - DNA, 45 bp, synthetic construct
  misc_feature 1..45: note = Description of Artificial Sequence: Synthetic oligonucleotide
  source 1..45: mol_type = other DNA
acttccaggctccacccgacgaaccccaaggggacctcatgcagg

SEQ ID NO: 142 - protein, 18 aa, Homo sapiens
LPGSTRLEGEPQGDLMQA

SEQ ID NO: 143 - DNA, 57 bp, Homo sapiens
  source 1..57: mol_type = other DNA
  CDS 2..55
acttccaggctccacccgactggagggcgaaccccaaggggacctcatgcaggctcc

SEQ ID NO: 144 - DNA, 46 bp, synthetic construct
  misc_feature 1..46: note = Description of Artificial Sequence: Synthetic oligonucleotide
  source 1..46: mol_type = other DNA
acttccaggctccacccgaaccccaaggggacctcatgcaggctcc

SEQ ID NO: 145 - DNA, 43 bp, synthetic construct
  misc_feature 1..43: note = Description of Artificial Sequence: Synthetic oligonucleotide
  source 1..43: mol_type = other DNA
acttccaggctccacccgaaccccaaggggacctcatgcaggc

SEQ ID NO: 146 - DNA, 20 bp, synthetic construct
  misc_feature 1..20: note = Description of Artificial Sequence: Synthetic oligonucleotide
  source 1..20: mol_type = other DNA
acttccaggctccacccgac

SEQ ID NO: 147 - DNA, 40 bp, synthetic construct
  misc_feature 1..40: note = Description of Artificial Sequence: Synthetic oligonucleotide
  source 1..40: mol_type = other DNA
acttccaggctccaccccaaggggacctcatgcaggctcc

SEQ ID NO: 148 - DNA, 58 bp, synthetic construct
  misc_feature 1..58: note = Description of Artificial Sequence: Synthetic oligonucleotide
  source 1..58: mol_type = other DNA
acttccaggctccacccgacttggagggcgaaccccaaggggacctcatgcaggctcc

SEQ ID NO: 149 - DNA, 46 bp, synthetic construct
  misc_feature 1..46: note = Description of Artificial Sequence: Synthetic oligonucleotide
  source 1..46: mol_type = other DNA
acttccaggctccaggcgaaccccaaggggacctcatgcaggctcc

SEQ ID NO: 150 - DNA, 32 bp, synthetic construct
  misc_feature 1..32: note = Description of Artificial Sequence: Synthetic oligonucleotide
  source 1..32: mol_type = other DNA
ggcgaaccccaaggggacctcatgcaggctcc

SEQ ID NO: 151 - DNA, 32 bp, synthetic construct
  misc_feature 1..32: note = Description of Artificial Sequence: Synthetic oligonucleotide
  source 1..32: mol_type = other DNA
acttccaggcaaggggacctcatgcaggctcc

SEQ ID NO: 152 - DNA, 33 bp, synthetic construct
  misc_feature 1..33: note = Description of Artificial Sequence: Synthetic oligonucleotide
  source 1..33: mol_type = other DNA
acttccaggctaaggggacctcatgcaggctcc

SEQ ID NO: 153 - DNA, 52 bp, Homo sapiens
  source 1..52: mol_type = other DNA
acttccaggctccacccgactggagggcgaaccccaaggggacctcatgcag

SEQ ID NO: 154 - DNA, 34 bp, synthetic construct
  misc_feature 1..34: note = Description of Artificial Sequence: Synthetic oligonucleotide
  source 1..34: mol_type = other DNA
acttccaggcgaaccccaaggggacctcatgcag

SEQ ID NO: 155 - DNA, 32 bp, synthetic construct
  misc_feature 1..32: note = Description of Artificial Sequence: Synthetic oligonucleotide
  source 1..32: mol_type = other DNA
acttccaggctccacaaggggacctcatgcag

SEQ ID NO: 156 - DNA, 34 bp, synthetic construct
  misc_feature 1..34: note = Description of Artificial Sequence: Synthetic oligonucleotide
  source 1..34: mol_type = other DNA
acttccaggctccacccaaggggacctcatgccc

SEQ ID NO: 157 - DNA, 35 bp, synthetic construct
  misc_feature 1..35: note = Description of Artificial Sequence: Synthetic oligonucleotide
  source 1..35: mol_type = other DNA
acttccaggctccaccccaaggggacctcatgcag

SEQ ID NO: 158 - DNA, 41 bp, synthetic construct
  misc_feature 1..41: note = Description of Artificial Sequence: Synthetic oligonucleotide
  source 1..41: mol_type = other DNA
acttccaggctccacccgaaccccaaggggacctcatgcag

SEQ ID NO: 159 - DNA, 50 bp, synthetic construct
  misc_feature 1..50: note = Description of Artificial Sequence: Synthetic oligonucleotide
  source 1..50: mol_type = other DNA
acttccaggctccacccgaaggagggcgaaccccaaggggacctcatgca

SEQ ID NO: 160 - DNA, 50 bp, synthetic construct
  misc_feature 1..50: note = Description of Artificial Sequence: Synthetic oligonucleotide
  source 1..50: mol_type = other DNA
acttccaggctccacccgactagggcgaaccccaaggggacctcatgcag

SEQ ID NO: 161 - DNA, 52 bp, synthetic construct
  misc_feature 1..52: note = Description of Artificial Sequence: Synthetic oligonucleotide
  source 1..52: mol_type = other DNA
acttccaggctccacccgactgggagggcgaaccccaaggggacctcatgca

SEQ ID NO: 162 - DNA, 52 bp, synthetic construct
  misc_feature 1..52: note = Description of Artificial Sequence: Synthetic oligonucleotide
  source 1..52: mol_type = other DNA
acttccaggctccacccgacttggagggcgaaccccaaggggacctcatgca

SEQ ID NO: 163 - DNA, 46 bp, synthetic construct
  misc_feature 1..46: note = Description of Artificial Sequence: Synthetic oligonucleotide
  source 1..46: mol_type = other DNA
acttccaggctccacccgaggcgaaccccaaggggacctcatgcag

SEQ ID NO: 164 - DNA, 47 bp, synthetic construct
  misc_feature 1..47: note = Description of Artificial Sequence: Synthetic oligonucleotide
  source 1..47: mol_type = other DNA
acttccaggctccacccgagggcgaaccccaaggggacctcatgcag

SEQ ID NO: 165 - DNA, 24 bp, synthetic construct
  misc_feature 1..24: note = Description of Artificial Sequence: Synthetic oligonucleotide
  source 1..24: mol_type = other DNA
acttccaggctccacctcatgcag

SEQ ID NO: 166 - DNA, 29 bp, synthetic construct
  misc_feature 1..29: note = Description of Artificial Sequence: Synthetic oligonucleotide
  source 1..29: mol_type = other DNA
agggcgaaccccaaggggacctcatgcag

SEQ ID NO: 167 - DNA, 45 bp, synthetic construct
  misc_feature 1..45: note = Description of Artificial Sequence: Synthetic oligonucleotide
  source 1..45: mol_type = other DNA
caatctatgacatcaattattatcggagccctgccaaaaaatcaa

SEQ ID NO: 168 - DNA, 45 bp, synthetic construct
  misc_feature 1..45: note = Description of Artificial Sequence: Synthetic oligonucleotide
  source 1..45: mol_type = other DNA
caatctatgacatcaattatcatcggagccctgccaaaaaatcaa

SEQ ID NO: 169 - DNA, 42 bp, synthetic construct
  misc_feature 1..42: note = Description of Artificial Sequence: Synthetic oligonucleotide
  source 1..42: mol_type = other DNA
caatctatgacatcaattatcggagccctgccaaaaaatcaa

SEQ ID NO: 170 - DNA, 48 bp, synthetic construct
  misc_feature 1..48: note = Description of Artificial Sequence: Synthetic oligonucleotide
  source 1..48: mol_type = other DNA
caatctatgacatcaattattatcatcggagccctgccaaaaaatcaa

SEQ ID NO: 171 - DNA, 33 bp, synthetic construct
  misc_feature 1..33: note = Description of Artificial Sequence: Synthetic oligonucleotide
  source 1..33: mol_type = other DNA
caatctatgacaagagccctgccaaaaaatcaa

SEQ ID NO: 172 - DNA, 52 bp, Homo sapiens
  source 1..52: mol_type = other DNA
ttctcaaggcagcatcatacttcccccacggtgggacagctgccctccctgg

SEQ ID NO: 173 - DNA, 46 bp, synthetic construct
  misc_feature 1..46: note = Description of Artificial Sequence: Synthetic oligonucleotide
  source 1..46: mol_type = other DNA
ttctcaaggcagcatcatacttccctgggacagctgccctccctgg

SEQ ID NO: 174 - DNA, 49 bp, synthetic construct
  misc_feature 1..49: note = Description of Artificial Sequence: Synthetic oligonucleotide
  source 1..49: mol_type = other DNA
ttctcaaggcagcatcatacttccacggtgggacagctgccctccctgg

SEQ ID NO: 175 - DNA, 25 bp, synthetic construct
  misc_feature 1..25: note = Description of Artificial Sequence: Synthetic oligonucleotide
  source 1..25: mol_type = other DNA
ttctcaaggcagctgccctccctgg

SEQ ID NO: 176 - DNA, 32 bp, synthetic construct
  misc_feature 1..32: note = Description of Artificial Sequence: Synthetic oligonucleotide
  source 1..32: mol_type = other DNA
ttctcaaggcagcatcatacttccctccctgg

SEQ ID NO: 177 - DNA, 264 bp, Homo sapiens
  modified_base 38..227: mod_base = OTHER; note = a, c, t, g, or unknown
  source 1..264: mol_type = other DNA
acaaagcgattttgaaagatggaagcgcggtggctatnnnnnnnnnnnnnnnnnnnnnnnnnnnnnnnnnnnnnnnnnnnnnnnnnnnnnnnnnnnnnnnnnnnnnnnnnnnnnnnnnnnnnnnnnnnnnnnnnnnnnnnnnnnnnnnnnnnnnnnnnnnnnnnnnnnnnnnnnnnnnnnnnnnnnnnnnnnnnnnnnnnnnnnnnnnnnnnnnnnnnnnnnnnnnnggggtgaaactaaactggtccacacggcggaagattg

SEQ ID NO: 178 - DNA, 257 bp, synthetic construct
  misc_feature 1..257: note = Description of Artificial Sequence: Synthetic polynucleotide
  modified_base 38..227: mod_base = OTHER; note = a, c, t, g, or unknown
  source 1..257: mol_type = other DNA
acaaagcgattttgaaagatggaagcgcggtggctatnnnnnnnnnnnnnnnnnnnnnnnnnnnnnnnnnnnnnnnnnnnnnnnnnnnnnnnnnnnnnnnnnnnnnnnnnnnnnnnnnnnnnnnnnnnnnnnnnnnnnnnnnnnnnnnnnnnnnnnnnnnnnnnnnnnnnnnnnnnnnnnnnnnnnnnnnnnnnnnnnnnnnnnnnnnnnnnnnnnnnnnnnnnnnnggggtgaaactaaaacacggcggaagattg

SEQ ID NO: 179 - DNA, 43 bp, synthetic construct
  misc_feature 1..43: note = Description of Artificial Sequence: Synthetic oligonucleotide
  source 1..43: mol_type = other DNA
acaaagcgattttgaaagatggaagcgacacggcggaagattg

SEQ ID NO: 180 - DNA, 44 bp, synthetic construct
  misc_feature 1..44: note = Description of Artificial Sequence: Synthetic oligonucleotide
  source 1..44: mol_type = other DNA
acaaagcgattttgaaagatggaagcgcacacggcggaagattg

SEQ ID NO: 181 - DNA, 106 bp, synthetic construct
  misc_feature 1..106: note = Description of Artificial Sequence: Synthetic polynucleotide
  source 1..106: mol_type = other DNA
acaaagcgattttgaaagatggaagcgaaatagcaagttaaaataaggctagtccgttatcaacttgaaaaagtggcaccgagtcggtgcacacggcggaagattg

SEQ ID NO: 182 - DNA, 23 bp, synthetic construct
  misc_feature 1..23: note = Description of Artificial Sequence: Synthetic oligonucleotide
  source 1..23: mol_type = other DNA
gggtggggggagtttgctcctgg

SEQ ID NO: 183 - DNA, 23 bp, synthetic construct
  misc_feature 1..23: note = Description of Artificial Sequence: Synthetic oligonucleotide
  source 1..23: mol_type = other DNA
ggatggagggagtttgctcctgg

SEQ ID NO: 184 - DNA, 23 bp, synthetic construct
  misc_feature 1..23: note = Description of Artificial Sequence: Synthetic oligonucleotide
  source 1..23: mol_type = other DNA
ggggaggggaagtttgctcctgg

SEQ ID NO: 185 - DNA, 23 bp, synthetic construct
  misc_feature 1..23: note = Description of Artificial Sequence: Synthetic oligonucleotide
  source 1..23: mol_type = other DNA
gaccccctccaccccgcctccgg

SEQ ID NO: 186 - DNA, 23 bp, synthetic construct
  misc_feature 1..23: note = Description of Artificial Sequence: Synthetic oligonucleotide
  source 1..23: mol_type = other DNA
gaccccccccaccccgcccccgg

SEQ ID NO: 187 - DNA, 23 bp, synthetic construct
  misc_feature 1..23: note = Description of Artificial Sequence: Synthetic oligonucleotide
  source 1..23: mol_type = other DNA
gcccccacccaccccgcctctgg

SEQ ID NO: 188 - DNA, 23 bp, synthetic construct
  misc_feature 1..23: note = Description of Artificial Sequence: Synthetic oligonucleotide
  source 1..23: mol_type = other DNA
ctccccacccaccccgcctcagg

SEQ ID NO: 189 - DNA, 23 bp, synthetic construct
  misc_feature 1..23: note = Description of Artificial Sequence: Synthetic oligonucleotide
  source 1..23: mol_type = other DNA
ggtgagtgagtgtgtgcgtgtgg

SEQ ID NO: 190 - DNA, 23 bp, synthetic construct
  misc_feature 1..23: note = Description of Artificial Sequence: Synthetic oligonucleotide
  source 1..23: mol_type = other DNA
tgtgggtgagtgtgtgcgtgagg

SEQ ID NO: 191 - DNA, 23 bp, synthetic construct
  misc_feature 1..23: note = Description of Artificial Sequence: Synthetic oligonucleotide
  source 1..23: mol_type = other DNA
gagtccgagcagaagaagaaggg

SEQ ID NO: 192 - DNA, 23 bp, synthetic construct
  misc_feature 1..23: note = Description of Artificial Sequence: Synthetic oligonucleotide
  source 1..23: mol_type = other DNA
gagttagagcagaagaagaaagg

SEQ ID NO: 193 - DNA, 23 bp, synthetic construct
  misc_feature 1..23: note = Description of Artificial Sequence: Synthetic oligonucleotide
  source 1..23: mol_type = other DNA
gaacctgagctgctctgacgcgg

SEQ ID NO: 194 - DNA, 23 bp, synthetic construct
  misc_feature 1..23: note = Description of Artificial Sequence: Synthetic oligonucleotide
  source 1..23: mol_type = other DNA
ttggcagggggtgggagggaagg

SEQ ID NO: 195 - DNA, 23 bp, synthetic construct
  misc_feature 1..23: note = Description of Artificial Sequence: Synthetic oligonucleotide
  source 1..23: mol_type = other DNA
gggagggagagcttggcaggggg

SEQ ID NO: 196 - DNA, 23 bp, synthetic construct
  misc_feature 1..23: note = Description of Artificial Sequence: Synthetic oligonucleotide
  source 1..23: mol_type = other DNA
gatggagccagagaggatcctgg

SEQ ID NO: 197 - DNA, 23 bp, synthetic construct
  misc_feature 1..23: note = Description of Artificial Sequence: Synthetic oligonucleotide
  source 1..23: mol_type = other DNA
cctgccaagctctccctcccagg

SEQ ID NO: 198 - DNA, 23 bp, synthetic construct
  misc_feature 1..23: note = Description of Artificial Sequence: Synthetic oligonucleotide
  source 1..23: mol_type = other DNA
ctccctcccaggatcctctctgg

SEQ ID NO: 199 - DNA, 23 bp, synthetic construct
  misc_feature 1..23: note = Description of Artificial Sequence: Synthetic oligonucleotide
  source 1..23: mol_type = other DNA
cctctaaggtttgcttacgatgg

SEQ ID NO: 200 - DNA, 23 bp, synthetic construct
  misc_feature 1..23: note = Description of Artificial Sequence: Synthetic oligonucleotide
  source 1..23: mol_type = other DNA
ggttctggcaaggagagagatgg

SEQ ID NO: 201 - DNA, 23 bp, synthetic construct
  misc_feature 1..23: note = Description of Artificial Sequence: Synthetic oligonucleotide
  source 1..23: mol_type = other DNA
tctaacccccacctcctgttagg

SEQ ID NO: 202 - DNA, 23 bp, synthetic construct
  misc_feature 1..23: note = Description of Artificial Sequence: Synthetic oligonucleotide
  source 1..23: mol_type = other DNA
ttggcagggggtgggagggatgg

SEQ ID NO: 203 - DNA, 23 bp, synthetic construct
  misc_feature 1..23: note = Description of Artificial Sequence: Synthetic oligonucleotide
  source 1..23: mol_type = other DNA
ttggtagggggtgggagggatgg

SEQ ID NO: 204 - DNA, 23 bp, synthetic construct
  misc_feature 1..23: note = Description of Artificial Sequence: Synthetic oligonucleotide
  source 1..23: mol_type = other DNA
gggaaggggagcttggcaggtgg

SEQ ID NO: 205 - DNA, 23 bp, synthetic construct
  misc_feature 1..23: note = Description of Artificial Sequence: Synthetic oligonucleotide
  source 1..23: mol_type = other DNA
ggtagtgagagcttggcaggtgg

SEQ ID NO: 206 - DNA, 23 bp, synthetic construct
  misc_feature 1..23: note = Description of Artificial Sequence: Synthetic oligonucleotide
  source 1..23: mol_type = other DNA
ctccctcccaggatcctcccagg

SEQ ID NO: 207 - DNA, 23 bp, synthetic construct
  misc_feature 1..23: note = Description of Artificial Sequence: Synthetic oligonucleotide
  source 1..23: mol_type = other DNA
gtccatggcaggatcctctcagg

SEQ ID NO: 208 - DNA, 23 bp, synthetic construct
  misc_feature 1..23: note = Description of Artificial Sequence: Synthetic oligonucleotide
  source 1..23: mol_type = other DNA
ctcccccccagtatcctctcagg

SEQ ID NO: 209 - DNA, 108 bp, Homo sapiens
  source 1..108: mol_type = other DNA
ccaatctatgacatcaattattatacatcggagccctgccaaaaaatcaatgtgaagcaaatcgcagcccgcctcctgcctccgctctactcactggtgttcatcttt

SEQ ID NO: 210 - DNA, 138 bp, Homo sapiens
  source 1..138: mol_type = other DNA
ccaccctataattctgaacctgcagaagaatctgaacataaaaacaacaattacgaaccaaacctatttaaaactccacaaaggaaaccatcttataatcagctggcttcaactccaataatattcaaagagcaaggg

SEQ ID NO: 211 - DNA, 121 bp, Homo sapiens
  misc_feature 49..50: note = Nucleotides at these positions are non-consecutive and are separated by a non-disclosed sequence
  source 1..121: mol_type = other DNA
ggccgggaatcaagagtcacccagagacagtgaccaaccatccctgtttagctctccctcccaggatcctctctggctccatcgtaagcaaaccttagaggttctggcaaggagagagatg

SEQ ID NO: 212 - DNA, 77 bp, synthetic construct
  misc_feature 1..77: note = Description of Artificial Sequence: Synthetic oligonucleotide
  source 1..77: mol_type = other DNA
ggccgggaatcaagagtcacccagtgaccaaccatccctgtaagcaaaccttagaggttctggcaaggagagagatg

SEQ ID NO: 213 - DNA, 27 bp, synthetic construct
  misc_feature 1..27: note = Description of Artificial Sequence: Synthetic oligonucleotide
  source 1..27: mol_type = other DNA
ggccgggaatcaagagtcacccaggaa

SEQ ID NO: 214 - DNA, 79 bp, synthetic construct
  misc_feature 1..79: note = Description of Artificial Sequence: Synthetic oligonucleotide
  source 1..79: mol_type = other DNA
ggccgggaatcaagagtcacccagacctctctggctccatcgtaagcaaaccttagaggttctggcaaggagagagatg

SEQ ID NO: 215 - DNA, 28 bp, synthetic construct
  misc_feature 1..28: note = Description of Artificial Sequence: Synthetic oligonucleotide
  source 1..28: mol_type = other DNA
ggccgggaatcaagagtcaccctaacag

SEQ ID NO: 216 - DNA, 66 bp, synthetic construct
  misc_feature 1..66: note = Description of Artificial Sequence: Synthetic oligonucleotide
  source 1..66: mol_type = other DNA
ggccgggaatcaagacgctggctccatcgtaagcaaaccttagaggttctggcaaggagagagatg

SEQ ID NO: 217 - DNA, 47 bp, synthetic construct
  misc_feature 1..47: note = Description of Artificial Sequence: Synthetic oligonucleotide
  source 1..47: mol_type = other DNA
ggctccatcgtaagcaaaccttagaggttctggcaaggagagagatg

SEQ ID NO: 218 - DNA, 78 bp, synthetic construct
  misc_feature 1..78: note = Description of Artificial Sequence: Synthetic oligonucleotide
  source 1..78: mol_type = other DNA
ggccgggaatcaagagtcacccagactctctggctccatcgtaagcaaaccttagaggttctggcaaggagagagatg

SEQ ID NO: 219 - DNA, 80 bp, synthetic construct
  misc_feature 1..80: note = Description of Artificial Sequence: Synthetic oligonucleotide
  source 1..80: mol_type = other DNA
ggccgggaatcaagagtcacccagagacagtgaccaaccatcgtaagcaaaccttagaggttctggcaaggagagagatg

SEQ ID NO: 220 - DNA, 46 bp, synthetic construct
  misc_feature 1..46: note = Description of Artificial Sequence: Synthetic oligonucleotide
  source 1..46: mol_type = other DNA
ggtccatcgtaagcaaaccttagaggttctggcaaggagagagatg

SEQ ID NO: 221 - DNA, 69 bp, synthetic construct
  misc_feature 1..69: note = Description of Artificial Sequence: Synthetic oligonucleotide
  source 1..69: mol_type = other DNA
ggccgggaatcaagagtcacccatctccatcgtaagcaaaccttagaggttctggcaaggagagagatg

SEQ ID NO: 222 - DNA, 76 bp, synthetic construct
  misc_feature 1..76: note = Description of Artificial Sequence: Synthetic oligonucleotide
  source 1..76: mol_type = other DNA
ggccgggaatcaagagtcacccagactctggctccatcgtaagcaaaccttagaggttctggcaaggagagagatg

SEQ ID NO: 223 - DNA, 50 bp, synthetic construct
  misc_feature 1..50: note = Description of Artificial Sequence: Synthetic oligonucleotide
  source 1..50: mol_type = other DNA
ggccgggaatcaagagtcacccagagacagtgaccaaccatcccatatca

SEQ ID NO: 224 - DNA, 59 bp, synthetic construct
  misc_feature 1..59: note = Description of Artificial Sequence: Synthetic oligonucleotide
  source 1..59: mol_type = other DNA
ggccgggaatcaagagtcatcgtaagcaaaccttagaggttctggcaaggagagagatg

SEQ ID NO: 225 - DNA, 24 bp, synthetic construct
  misc_feature 1..24: note = Description of Artificial Sequence: Synthetic oligonucleotide
  source 1..24: mol_type = other DNA
aatgaccactacatccttcaaggg

SEQ ID NO: 226 - DNA, 25 bp, synthetic construct
  misc_feature 1..25: note = Description of Artificial Sequence: Synthetic oligonucleotide
  source 1..25: mol_type = other DNA
aatgaccactacatcctttcaaggg

SEQ ID NO: 227 - DNA, 26 bp, synthetic construct
  misc_feature 1..26: note = Description of Artificial Sequence: Synthetic oligonucleotide
  source 1..26: mol_type = other DNA
aatgaccactacatccttttcaaggg

SEQ ID NO: 228 - DNA, 22 bp, synthetic construct
  misc_feature 1..22: note = Description of Artificial Sequence: Synthetic oligonucleotide
  source 1..22: mol_type = other DNA
aatgaccactacatcctaaggg

SEQ ID NO: 229 - DNA, 21 bp, synthetic construct
  misc_feature 1..21: note = Description of Artificial Sequence: Synthetic oligonucleotide
  source 1..21: mol_type = other DNA
aatgaccactacatcctaggg

SEQ ID NO: 230 - DNA, 20 bp, synthetic construct
  misc_feature 1..20: note = Description of Artificial Sequence: Synthetic oligonucleotide
  source 1..20: mol_type = other DNA
aatgaccactacatcctggg

SEQ ID NO: 231 - DNA, 42 bp, Homo sapiens
  source 1..42: mol_type = other DNA
tatgtgcaatgaccactacatcctcaagggcagcaatcggag

SEQ ID NO: 232 - DNA, 45 bp, synthetic construct
  misc_feature 1..45: note = Description of Artificial Sequence: Synthetic oligonucleotide
  source 1..45: mol_type = other DNA
tatgtgcaatgaccactacatcctcctcaagggcagcaatcggag

SEQ ID NO: 233 - DNA, 30 bp, synthetic construct
  misc_feature 1..30: note = Description of Artificial Sequence: Synthetic oligonucleotide
  source 1..30: mol_type = other DNA
tatgtgcaatgaccactacatcaatcggag

SEQ ID NO: 234 - DNA, 33 bp, synthetic construct
  misc_feature 1..33: note = Description of Artificial Sequence: Synthetic oligonucleotide
  source 1..33: mol_type = other DNA
tatgtgcaatgaccactacatcagcaatcggag

SEQ ID NO: 235 - DNA, 34 bp, synthetic construct
  misc_feature 1..34: note = Description of Artificial Sequence: Synthetic oligonucleotide
  source 1..34: mol_type = other DNA
tatgtgcaatgaccactacatccagcaatcggag

SEQ ID NO: 236 - DNA, 10 bp, synthetic construct
  misc_feature 1..10: note = Description of Artificial Sequence: Synthetic oligonucleotide
  source 1..10: mol_type = other DNA
cagcaatcgg

SEQ ID NO: 237 - DNA, 41 bp, synthetic construct
  misc_feature 1..41: note = Description of Artificial Sequence: Synthetic oligonucleotide
  source 1..41: mol_type = other DNA
tatgtgcaatgaccactacatccttcaagggcagcaatcgg

SEQ ID NO: 238 - DNA, 41 bp, synthetic construct
  misc_feature 1..41: note = Description of Artificial Sequence: Synthetic oligonucleotide
  source 1..41: mol_type = other DNA
tatgtgcaatgaccactacatcctccaagggcagcaatcgg

SEQ ID NO: 239 - DNA, 41 bp, synthetic construct
  misc_feature 1..41: note = Description of Artificial Sequence: Synthetic oligonucleotide
  source 1..41: mol_type = other DNA
tatgtgcaatgaccactacatcctbcaagggcagcaatcgg

SEQ ID NO: 240 - DNA, 34 bp, synthetic construct
  misc_feature 1..34: note = Description of Artificial Sequence: Synthetic oligonucleotide
  source 1..34: mol_type = other DNA
tatgtgcaatgaccactacattggcagcaatcgg

SEQ ID NO: 241 - DNA, 21 bp, synthetic construct
  misc_feature 1..21: note = Description of Artificial Sequence: Synthetic oligonucleotide
  source 1..21: mol_type = other DNA
tatgtgcaatgaccactacat

SEQ ID NO: 242 - DNA, 53 bp, Homo sapiens
  source 1..53: mol_type = other DNA
tcatacagatgatgtctcatcatcagaggagcgagaaggtaaagtcaaaatca

SEQ ID NO: 243 - DNA, 32 bp, synthetic construct
  misc_feature 1..32: note = Description of Artificial Sequence: Synthetic oligonucleotide
  source 1..32: mol_type = other DNA
tcatacagatgatacaggtaaagtcaaaatca

SEQ ID NO: 244 - DNA, 32 bp, synthetic construct
  misc_feature 1..32: note = Description of Artificial Sequence: Synthetic oligonucleotide
  source 1..32: mol_type = other DNA
tcatacaggtgatgaaggtaaagtcaaaatca

SEQ ID NO: 245 - DNA, 50 bp, synthetic construct
  misc_feature 1..50: note = Description of Artificial Sequence: Synthetic oligonucleotide
  source 1..50: mol_type = other DNA
tcatacagatgatgtctcatcatcagagcgagaaggtaaagtcaaaatca

SEQ ID NO: 246 - DNA, 48 bp, synthetic construct
  misc_feature 1..48: note = Description of Artificial Sequence: Synthetic oligonucleotide
  source 1..48: mol_type = other DNA
tcatacagatgatgtctcatcatcagcgagaaggtaaagtcaaaatca

SEQ ID NO: 247 - DNA, 52 bp, synthetic construct
  misc_feature 1..52: note = Description of Artificial Sequence: Synthetic oligonucleotide
  source 1..52: mol_type = other DNA
tcatacagatgatgtctcatcatcagggagcgagaaggtaaagtcaaaatca

SEQ ID NO: 248 - DNA, 41 bp, synthetic construct
  misc_feature 1..41: note = Description of Artificial Sequence: Synthetic oligonucleotide
  source 1..41: mol_type = other DNA
tcatacagatgatgtctcgcgagaaggtaaagtcaaaatca

SEQ ID NO: 249 - DNA, 32 bp, synthetic construct
  misc_feature 1..32: note = Description of Artificial Sequence: Synthetic oligonucleotide
  source 1..32: mol_type = other DNA
tcatacagatgatgaaggtaaagtcaaaatca

SEQ ID NO: 250 - DNA, 29 bp, synthetic construct
  misc_feature 1..29: note = Description of Artificial Sequence: Synthetic oligonucleotide
  source 1..29: mol_type = other DNA
tcatacagatgaaggtaaagtcaaaatca

SEQ ID NO: 251 - DNA, 42 bp, synthetic construct
  misc_feature 1..42: note = Description of Artificial Sequence: Synthetic oligonucleotide
  source 1..42: mol_type = other DNA
tcatacagatgatgtctacagatgaaggtaaagtcaaaatca

SEQ ID NO: 252 - DNA, 51 bp, synthetic construct
  misc_feature 1..51: note = Description of Artificial Sequence: Synthetic oligonucleotide
  source 1..51: mol_type = other DNA
tcatacagatgatgtctcatcatcaggagcgagaaggtaaagtcaaaatca

SEQ ID NO: 253 - DNA, 34 bp, synthetic construct
  misc_feature 1..34: note = Description of Artificial Sequence: Synthetic oligonucleotide
  source 1..34: mol_type = other DNA
gtcatcctcatcctgataaactgcaaaaggctga

SEQ ID NO: 254 - DNA, 606 bp, Homo sapiens
  source 1..606: mol_type = other DNA
gctggtgtctgggttctgtgccccttccccaccccagcccaccccaggtgtcctgtccattctcaggctggtcacatgggtggtcctagggtgtcccatgagagatgcaaagcgcctgaattttctgactcttcccatcagaccccccaaagacacatgtgacccaccaccccatctctgaccatgaggccaccctgaggtgctgggccctgggcttctaccctgcggagatcacactgacctggcagcgggatggcgaggaccaaactcaggacaccgagcttgtggagaccagaccagcaggagatagaaccttccagaagtgggcagctgtggtggtgccttctggagaagagcagagatacacatgccatgtacagcatgaggggctgccgaagcccctcaccctgagatggggtaaggagggggatgaggggtcatatctgttcatatctgttctcagggaaagcaggagcccttctggagcccttcagcagggtcagggcccctcatcttcccctcctttcccagagccatcttcccagtccaccatccccatcgtgggcattgttgctggcctggctgtcctagcagttgtggtcatcg

SEQ ID NO: 255 - DNA, 26 bp, Homo sapiens
  source 1..26: mol_type = other DNA
actaccacagctccttctctgagtgg

SEQ ID NO: 256 - DNA, 23 bp, synthetic construct
  misc_feature 1..23: note = Description of Artificial Sequence: Synthetic oligonucleotide
  source 1..23: mol_type = other DNA
actaccacagctcctctgagtgg

SEQ ID NO: 257 - DNA, 23 bp, Homo sapiens
  source 1..23: mol_type = other DNA
gtagttggagctggcggcgtagg

SEQ ID NO: 258 - DNA, 23 bp, synthetic construct
  misc_feature 1..23: note = Description of Artificial Sequence: Synthetic oligonucleotide
  source 1..23: mol_type = other DNA
gtagttggagctagcggcgtagg

SEQ ID NO: 259 - DNA, 23 bp, Homo sapiens
  source 1..23: mol_type = other DNA
gtagttggagctggtggcgtagg

SEQ ID NO: 260 - DNA, 23 bp, synthetic construct
  misc_feature 1..23: note = Description of Artificial Sequence: Synthetic oligonucleotide
  source 1..23: mol_type = other DNA
gtagttggagctagtggcgtagg

SEQ ID NO: 261 - DNA, 28 bp, synthetic construct
  misc_feature 1..28: note = Description of Artificial Sequence: Synthetic oligonucleotide
  source 1..28: mol_type = other DNA
ccatacattaaagatagtcatcttgggg

SEQ ID NO: 262 - DNA, 60 bp, Homo sapiens
  source 1..60: mol_type = other DNA
ccatacagtcagtatcaattctggaagaatttccagacattaaagatagtcatcttgggg

SEQ ID NO: 263 - DNA, 55 bp, Homo sapiens
  source 1..55: mol_type = other DNA
ccatacagtcagtatcaattctggaagaatttccagacattaaagatagtcatct

SEQ ID NO: 264 - DNA, 23 bp, synthetic construct
  misc_feature 1..23: note = Description of Artificial Sequence: Synthetic oligonucleotide
  source 1..23: mol_type = other DNA
ccatacattaaagatagtcatct

SEQ ID NO: 265 - DNA, 23 bp, Homo sapiens
  source 1..23: mol_type = other DNA
agatgactatctttaatgtctgg

SEQ ID NO: 266 - DNA, 23 bp, Homo sapiens
  source 1..23: mol_type = other DNA
agatgactatctttaatgtatgg

SEQ ID NO: 267 - DNA, 23 bp, synthetic construct
  misc_feature 1..23: note = Description of Artificial Sequence: Synthetic oligonucleotide
  source 1..23: mol_type = other DNA
gtagttggagctgatggcgtagg

SEQ ID NO: 268 - DNA, 23 bp, synthetic construct
  misc_feature 1..23: note = Description of Artificial Sequence: Synthetic oligonucleotide
  source 1..23: mol_type = other DNA
gtagttggagctggtagcgtagg

SEQ ID NO: 269 - DNA, 23 bp, synthetic construct
  misc_feature 1..23: note = Description of Artificial Sequence: Synthetic oligonucleotide
  source 1..23: mol_type = other DNA
gtagttggagctggtgacgtagg

SEQ ID NO: 270 - DNA, 23 bp, synthetic construct
  misc_feature 1..23: note = Description of Artificial Sequence: Synthetic oligonucleotide
  source 1..23: mol_type = other DNA
gtagttggagctaatggcgtagg

SEQ ID NO: 271 - DNA, 23 bp, synthetic construct
  misc_feature 1..23: note = Description of Artificial Sequence: Synthetic oligonucleotide
  source 1..23: mol_type = other DNA
gtagttggagctagtagcgtagg

SEQ ID NO: 272 - DNA, 23 bp, synthetic construct
  misc_feature 1..23: note = Description of Artificial Sequence: Synthetic oligonucleotide
  source 1..23: mol_type = other DNA
gtagttggagctagtgacgtagg

SEQ ID NO: 273 - DNA, 23 bp, Homo sapiens
  source 1..23: mol_type = other DNA
caaatgaatgatgcacatcatgg

SEQ ID NO: 274 - DNA, 23 bp, synthetic construct
  misc_feature 1..23: note = Description of Artificial Sequence: Synthetic oligonucleotide
  source 1..23: mol_type = other DNA
caaatgaatgatgcacgtcatgg

SEQ ID NO: 275 - DNA, 23 bp, synthetic construct
  misc_feature 1..23: note = Description of Artificial Sequence: Synthetic oligonucleotide
  source 1..23: mol_type = other DNA
caaatgaatgatgcatatcatgg

SEQ ID NO: 276 - DNA, 23 bp, synthetic construct
  misc_feature 1..23: note = Description of Artificial Sequence: Synthetic oligonucleotide
  source 1..23: mol_type = other DNA
caaatgaatgatgcgcatcatgg

SEQ ID NO: 277 - DNA, 23 bp, synthetic construct
  misc_feature 1..23: note = Description of Artificial Sequence: Synthetic oligonucleotide
  source 1..23: mol_type = other DNA
caaatgaatgatgtacatcatgg

SEQ ID NO: 278 - DNA, 23 bp, synthetic construct
  misc_feature 1..23: note = Description of Artificial Sequence: Synthetic oligonucleotide
  source 1..23: mol_type = other DNA
caaatgaatggtgcacatcatgg

SEQ ID NO: 279 - DNA, 23 bp, synthetic construct
  misc_feature 1..23: note = Description of Artificial Sequence: Synthetic oligonucleotide
  source 1..23: mol_type = other DNA
caaatgagtgatgcacatcatgg

SEQ ID NO: 280 - DNA, 23 bp, synthetic construct
  misc_feature 1..23: note = Description of Artificial Sequence: Synthetic oligonucleotide
  source 1..23: mol_type = other DNA
caaaagaatgatgcacatcatgg

SEQ ID NO: 281 - DNA, 23 bp, synthetic construct
  misc_feature 1..23: note = Description of Artificial Sequence: Synthetic oligonucleotide
  source 1..23: mol_type = other DNA
cgaatgaatgatgcacatcatgg

SEQ ID NO: 282 - DNA, 23 bp, synthetic construct
  misc_feature 1..23: note = Description of Artificial Sequence: Synthetic oligonucleotide
  source 1..23: mol_type = other DNA
caaatgaatgatgcatgtcatgg

SEQ ID NO: 283 - DNA, 23 bp, synthetic construct
  misc_feature 1..23: note = Description of Artificial Sequence: Synthetic oligonucleotide
  source 1..23: mol_type = other DNA
caaatgaatgatgcgcgtcatgg

SEQ ID NO: 284 - DNA, 23 bp, synthetic construct
  misc_feature 1..23: note = Description of Artificial Sequence: Synthetic oligonucleotide
  source 1..23: mol_type = other DNA
caaatgaatgatgtacgtcatgg

SEQ ID NO: 285 - DNA, 23 bp, synthetic construct
  misc_feature 1..23: note = Description of Artificial Sequence: Synthetic oligonucleotide
  source 1..23: mol_type = other DNA
caaatgaatggtgcacgtcatgg

SEQ ID NO: 286 - DNA, 23 bp, synthetic construct
  misc_feature 1..23: note = Description of Artificial Sequence: Synthetic oligonucleotide
  source 1..23: mol_type = other DNA
caaatgagtgatgcacgtcatgg

SEQ ID NO: 287 - DNA, 23 bp, synthetic construct
  misc_feature 1..23: note = Description of Artificial Sequence: Synthetic oligonucleotide
  source 1..23: mol_type = other DNA
caaaagaatgatgcacgtcatgg

SEQ ID NO: 288 - DNA, 23 bp, synthetic construct
  misc_feature 1..23: note = Description of Artificial Sequence: Synthetic oligonucleotide
  source 1..23: mol_type = other DNA
cgaatgaatgatgcacgtcatgg

SEQ ID NO: 289 - DNA, 23 bp, Homo sapiens
  source 1..23: mol_type = other DNA
atcataggtcgtcatgcttatgg

SEQ ID NO: 290 - DNA, 23 bp, synthetic construct
  misc_feature 1..23: note = Description of Artificial Sequence: Synthetic oligonucleotide
  source 1..23: mol_type = other DNA
atcataggttgtcatgcttatgg

SEQ ID NO: 291 - DNA, 23 bp, Homo sapiens
  source 1..23: mol_type = other DNA
atcataggtcgtcctgcttatgg

SEQ ID NO: 292 - DNA, 23 bp, synthetic construct
  misc_feature 1..23: note = Description of Artificial Sequence: Synthetic oligonucleotide
  source 1..23: mol_type = other DNA
atcataggttgtcctgcttatgg

SEQ ID NO: 293 - DNA, 23 bp, Homo sapiens
  source 1..23: mol_type = other DNA
ctggacaagaagagtacagtgcc

SEQ ID NO: 294 - DNA, 23 bp, synthetic construct
  misc_feature 1..23: note = Description of Artificial Sequence: Synthetic oligonucleotide
  source 1..23: mol_type = other DNA
ctggaaaagaagagtacagtgcc

SEQ ID NO: 295 - DNA, 23 bp, Homo sapiens
  source 1..23: mol_type = other DNA
actccatcgagatttcactgtag

SEQ ID NO: 296 - DNA, 23 bp, synthetic construct
  misc_feature 1..23: note = Description of Artificial Sequence: Synthetic oligonucleotide
  source 1..23: mol_type = other DNA
actccatcgagatttctctgtag